European Patent Specification EP 3 331 912 B1, published May 1, 2024. Title: INSERTABLE VARIABLE FRAGMENTS OF ANTIBODIES AND MODIFIED ALPHA1-ALPHA2 DOMAINS OF NKG2D LIGANDS, AND NON-NATURAL NKG2D LIGANDS THAT BIND NON-NATURAL NKG2D RECEPTORS. Applicant: AvidBiotics Corp. The sequence listing filed with the application follows.

SEQUENCE LISTING (105 sequences)

SEQ ID NO: 1 - DNA, 1126 bp, Artificial Sequence
  Synthetic polynucleotide, encoding alpha3-iFv.1
ccccccatggtgcaagttacccgcagcgaggcctcaggagatcgcgtaactatcacttgcagagcttctcaggacgtgtccaccgcggttgcttggtaccagcaaaagcctggaaaggcgccgaagctgctgatctactccgcctcattcttgtactcaggagtgcccagtcgatttagtggtagcggttctggtactgatttcacccttaccatcagcagtctccagcccgaggatttcgctacttattactgccagcagtcatacaccactcctcccactttcggccaaggtaccaaggtcgagattaaaggcggaagctctaggtcctctagctccggaggaggtggctctggcggcggcggagaagtccaactggtggagagcggaggcggactggtgcagccaggcggatccttgagacttagctgtgcggcttcgggttttacctttacttctactggcatcagttgggtcagacaagcgcctggcaagggactggaatgggttggacgtatctaccccactaatggttcgacgaactatgcggatagtgtgaaaggtagattcacgatatctgctgacacctcgaagaataccgcttaccttcaaatgaatagtttgcgtgccgaagatactgctgtctactattgcgccagaacctatggaatatacgacctttatgtggactacaccgagtacgtcatggattattggggccagggtacgttggtgacagtgtcgagtggcggaagctctaggtcctctagctccggaggaggtggctctggcggcggcggagacattcagatgactcagtctcccagttctcttagtgcctctggccaaattaccgtcacgtgtcgtgctagcggcttctacccgtggaatatcaccctgagctggcgccaagacggtgttagcctgagccacgacacccaacaatggggcgacgtgttgccagatggccaaggtacctaccagacgtgggttgccacccgtatttcccagggtgaagagcagcgttttacctgctatatggaacacagcggccaacatagcacgcatccggtgccgagcggtaaaggtagccaccatcatcaccaccattagtaggaattccgga

SEQ ID NO: 2 - DNA, 1144 bp, Artificial Sequence
  Synthetic polynucleotide, encoding alpha3-iFv.2
ccccccatggtgcaagttacccgcagcgaggcctcaggcggaagcggagatcgcgtaactatcacttgcagagcttctcaggacgtgtccaccgcggttgcttggtaccagcaaaagcctggaaaggcgccgaagctgctgatctactccgcctcattcttgtactcaggagtgcccagtcgatttagtggtagcggttctggtactgatttcacccttaccatcagcagtctccagcccgaggatttcgctacttattactgccagcagtcatacaccactcctcccactttcggccaaggtaccaaggtcgagattaaaggcggaagctctaggtcctctagctccggaggaggtggctctggcggcggcggagaagtccaactggtggagagcggaggcggactggtgcagccaggcggatccttgagacttagctgtgcggcttcgggttttacctttacttctactggcatcagttgggtcagacaagcgcctggcaagggactggaatgggttggacgtatctaccccactaatggttcgacgaactatgcggatagtgtgaaaggtagattcacgatatctgctgacacctcgaagaataccgcttaccttcaaatgaatagtttgcgtgccgaagatactgctgtctactattgcgccagaacctatggaatatacgacctttatgtggactacaccgagtacgtcatggattattggggccagggtacgttggtgacagtgtcgagtggcggaagctctaggtcctctagctccggaggaggtggctctggcggcggcggagacattcagatgactcagtctcccagttctcttagtgcctctggcggaagcggccaaattaccgtcacgtgtcgtgctagcggcttctacccgtggaatatcaccctgagctggcgccaagacggtgttagcctgagccacgacacccaacaatggggcgacgtgttgccagatggccaaggtacctaccagacgtgggttgccacccgtatttcccagggtgaagagcagcgttttacctgctatatggaacacagcggccaacatagcacgcatccggtgccgagcggtaaaggtagccaccatcatcaccaccattagtaggaattccgga

SEQ ID NO: 3 - protein, 269 aa, Artificial Sequence
  Synthetic peptide iFv (fgfr3)
GDRVTITCRASQDVSTAVAWYQQKPGKAPKLLIYSASFLYSGVPSRFSGSGSGTDFTLTISSLQPEDFATYYCQQSYTTPPTFGQGTKVEIKGGSSRSSSSGGGGSGGGGEVQLVESGGGLVQPGGSLRLSCAASGFTFTSTGISWVRQAPGKGLEWVGRIYPTNGSTNYADSVKGRFTISADTSKNTAYLQMNSLRAEDTAVYYCARTYGIYDLYVDYTEYVMDYWGQGTLVTVSSGGSSRSSSSGGGGSGGGGDIQMTQSPSSLSAS

SEQ ID NO: 4 - DNA, 807 bp, Artificial Sequence
  Synthetic polynucleotide, encoding iFv (fgfr3)
ggagatcgcgtaactatcacttgcagagcttctcaggacgtgtccaccgcggttgcttggtaccagcaaaagcctggaaaggcgccgaagctgctgatctactccgcctcattcttgtactcaggagtgcccagtcgatttagtggtagcggttctggtactgatttcacccttaccatcagcagtctccagcccgaggatttcgctacttattactgccagcagtcatacaccactcctcccactttcggccaaggtaccaaggtcgagattaaaggcggaagctctaggtcctctagctccggaggaggtggctctggcggcggcggagaagtccaactggtggagagcggaggcggactggtgcagccaggcggatccttgagacttagctgtgcggcttcgggttttacctttacttctactggcatcagttgggtcagacaagcgcctggcaagggactggaatgggttggacgtatctaccccactaatggttcgacgaactatgcggatagtgtgaaaggtagattcacgatatctgctgacacctcgaagaataccgcttaccttcaaatgaatagtttgcgtgccgaagatactgctgtctactattgcgccagaacctatggaatatacgacctttatgtggactacaccgagtacgtcatggattattggggccagggtacgttggtgacagtgtcgagtggcggaagctctaggtcctctagctccggaggaggtggctctggcggcggcggagacattcagatgactcagtctcccagttctcttagtgcctct

SEQ ID NO: 5 - protein, 18 aa, Artificial Sequence
  Synthetic peptide linker region
GGSSRSSSSGGGGSGGGG

SEQ ID NO: 6 - protein, 370 aa, Artificial Sequence
  Synthetic peptide alpha3-iFv.1
PPMVQVTRSEASGDRVTITCRASQDVSTAVAWYQQKPGKAPKLLIYSASFLYSGVPSRFSGSGSGTDFTLTISSLQPEDFATYYCQQSYTTPPTFGQGTKVEIKGGSSRSSSSGGGGSGGGGEVQLVESGGGLVQPGGSLRLSCAASGFTFTSTGISWVRQAPGKGLEWVGRIYPTNGSTNYADSVKGRFTISADTSKNTAYLQMNSLRAEDTAVYYCARTYGIYDLYVDYTEYVMDYWGQGTLVTVSSGGSSRSSSSGGGGSGGGGDIQMTQSPSSLSASGQITVTCRASGFYPWNITLSWRQDGVSLSHDTQQWGDVLPDGQGTYQTWVATRISQGEEQRFTCYMEHSGQHSTHPVPSGKGSHHHHHH

SEQ ID NO: 7 - protein, 376 aa, Artificial Sequence
  Synthetic peptide alpha3-iFv.2
PPMVQVTRSEASGGSGDRVTITCRASQDVSTAVAWYQQKPGKAPKLLIYSASFLYSGVPSRFSGSGSGTDFTLTISSLQPEDFATYYCQQSYTTPPTFGQGTKVEIKGGSSRSSSSGGGGSGGGGEVQLVESGGGLVQPGGSLRLSCAASGFTFTSTGISWVRQAPGKGLEWVGRIYPTNGSTNYADSVKGRFTISADTSKNTAYLQMNSLRAEDTAVYYCARTYGIYDLYVDYTEYVMDYWGQGTLVTVSSGGSSRSSSSGGGGSGGGGDIQMTQSPSSLSASGGSGQITVTCRASGFYPWNITLSWRQDGVSLSHDTQQWGDVLPDGQGTYQTWVATRISQGEEQRFTCYMEHSGQHSTHPVPSGKGSHHHHHH

SEQ ID NO: 8 - protein, 368 aa, Artificial Sequence
  Synthetic peptide alpha3-iFv.3(CD20)
PPMVQVTRSEASGGSGEKVTMTCRASSSVSYIHWFQQKPGSSPKPWIYATSNLASGVPVRFSGSGSGTSYSLTISRVEAEDAATYYCQQWTSNPPTFGGGTKLEIKGGSSRSSSSGGGGSGGGGQVQLQQPGAELVKPGASVKMSCKASGYTFTSYNMHWVKQTPGRGLEWIGAIYPGNGDTSYNQKFKGKATLTADKSSSTAYMQLSSLTSEDSAVYYCARSTYYGGDWYFNVWGAGTTVTVSAGGSSRSSSSGGGGSGGGGQIVLSQSPAILSASGGSQITVTCRASGFYPWNITLSWRQDGVSLSHDTQQWGDVLPDGQGTYQTWVATRISQGEEQRFTCYMEHSGQHSTHPVPSGKGSHHHHHH

SEQ ID NO: 9 - DNA, 561 bp, Artificial Sequence
  Synthetic polynucleotide, encoding ULBP1 alpha1-alpha2
gctgctgagccccactgtctctgctacgactttattataactcctaagtcaagaccagagcctcagtggtgcgaagtacaaggtttggttgacgaaaggcctttccttcactacgattgtgtgaaccataaggcaaaggctttcgccagcctgggtaagaaggtaaacgttactaagacgtgggaggagcagacggaaaccctccgtgatgtggttgactttcttaagggtcagctcctcgatatccaagtggagaatttaatccctatcgaaccgctcactctgcaggccagaatgtcatgcgaacatgaagcacacggtcatggaagaggtagttggcaatttttatttaacggtcaaaaattcctgctgttcgactcaaacaaccgcaaatggactgcgctgcaccctggagctaagaagatgactgaaaaatgggagaagaacagagacgttaccatgttcttccagaagatttccctgggagattgtaagatgtggttagaggagttcttaatgtactgggaacagatgctggaccccacaaaaccccccatggtg

SEQ ID NO: 10 - DNA, 567 bp, Artificial Sequence
  Synthetic polynucleotide, encoding ULBP2 alpha1-alpha2
gctgctgagccccatagtctgtgttacgacatcacagttattcccaagttcaggcccggaccgcgctggtgtgccgtgcaaggacaagtcgacgaaaaaacctttcttcattacgattgcggaaataagactgtaacgccagtctctcctttaggtaagaagttaaacgtcactacggcgtggaaggcacaaaaccccgtcctgcgcgaggtcgtcgacatcctgactgaacaattgcgcgacatccagctcgagaattacactccaaaggagcctcttaccctgcaggctagaatgtcttgcgagcaaaaggcagagggccactcctccggcagctggcagttcagtttcgacggacaaatctttctgttattcgattcagagaagagaatgtggactacagttcaccccggtgcccgtaaaatgaaggagaagtgggaaaacgacaaagtggtggcgatgtcattccactatttctcgatgggagactgcatcggttggctggaagatttcctcatgggtatggactccactttggagccatcggctggtgccccccccatggtg

SEQ ID NO: 11 - DNA, 561 bp, Artificial Sequence
  Synthetic polynucleotide, encoding ULBP3 alpha1-alpha2
gctgctgagccccacagcttgtggtacaacttcaccattatccacttgccgagacatggccagcagtggtgcgaagtgcaatcgcaagtcgaccaaaaaaacttcttatcatacgactgcggcagcgataaggtcttatctatgggtcatttggaggaacagctctacgcgaccgacgcctggggtaaacagctcgagatgctccgtgaggttggacagaggctgagactggaactggctgacactgagctggaagatttcacacctagtggtccactcacattgcaagtacgcatgagctgcgagtgtgaggccgatggatacattaggggcagctggcagtttagcttcgacggaaggaaattcctgctcttcgacagtaacaataggaagtggactgttgtgcatgctggtgcgcgcagaatgaaggaaaagtgggagaaagatagcggcctgacgaccttcttcaagatggtgtctatgcgtgactgtaagagctggctcagagatttcctcatgcatcgcaagaagaggttagaacctaccgctccccccatggtg

SEQ ID NO: 12 - DNA, 561 bp, Artificial Sequence
  Synthetic polynucleotide, encoding ULBP4 alpha1-alpha2
gctgctgagccccactctctttgcttcaacttcaccattaaatccctgagcaggcctggtcagccgtggtgtgaggcgcaggtctttcttaacaagaatctcttcctccaatacaactctgataacaacatggtaaagccactgggtctcctgggtaaaaaagtctatgctacgagcacttggggagaactcacccagactcttggcgaggtaggaagagacctgcgcatgctcctctgcgatataaagccccaaattaagaccagtgatccgtccactttacaagtcgaaatgttctgccaaagggaggctgaacgctgcaccggagcctcttggcagttcgcgaccaatggcgaaaagtccctcttgttcgatgccatgaatatgacctggaccgtgatcaatcatgaggcctctaagatcaaggagacgtggaaaaaggaccgcggccttgaaaagtactttaggaagttgtctaaaggagactgcgaccattggttacgcgagttcctcggccattgggaagcgatgcccgagccaacggttagcccccccatggtg

SEQ ID NO: 13 - DNA, 567 bp, Artificial Sequence
  Synthetic polynucleotide, encoding ULBP6 alpha1-alpha2
gctgctgagccccactccttatgctatgatatcaccgtgattccaaagttccgaccaggaccccgatggtgcgccgtacagggacaggtcgacgaaaagacttttttacattacgactgcggtaacaagacagtcacaccggtaagtcctttgggaaaaaagttaaacgtaaccactgcttggaaggcccagaaccccgtccttcgagaagtagtggatattttgactgaacagctgcttgacatccagctggaaaactacacacccaaagagcccctgactcttcaagcgcgtatgtcgtgtgagcaaaaggccgaaggacacagctccggatcctggcagttcagtatcgacggtcagaccttcctcctcttcgattcagaaaagcgcatgtggactactgtgcaccccggcgctcgtaagatgaaggaaaagtgggagaatgataaggacgttgccatgagttttcattacattagtatgggagattgcatcggttggctggaagacttcctgatgggtatggatagtacccttgaacctagtgccggagctccccccatggtg

SEQ ID NO: 14 - DNA, 483 bp, Artificial Sequence
  Synthetic polynucleotide, encoding OMCP alpha1-alpha2
gctgctgctgagccccacaagcttgcgttcaacttcaatctggaaataaacggttcagatacccattcaaccgtggacgtttatttagacgattcgcagataatcacctttgacggcaaggacatccgcccaactatcccgttcatgataggtgacgaaatcttccttcctttttataagaatgtgttctctgagttcttcagtttgttccgccgcgtccctacctcaaccccctacgaagacttgacttatttctatgaatgcgactacaccgacaacaaatctacattcgatcaattctacctgtacaacggtgaagagtacaccgtgaagactcaagaggctactaacaagaacatgtggctgaccacttccgagttcagactgaagaagtggttcgacggcgaggactgtatcatgcaccttagaagtttagtgaggaaaatggaagatagcaagagaagaacagtgccccccatggtg

SEQ ID NO: 15 - protein, 187 aa, Artificial Sequence
  Synthetic peptide ULBP1 alpha1-alpha2
AAEPHCLCYDFIITPKSRPEPQWCEVQGLVDERPFLHYDCVNHKAKAFASLGKKVNVTKTWEEQTETLRDVVDFLKGQLLDIQVENLIPIEPLTLQARMSCEHEAHGHGRGSWQFLFNGQKFLLFDSNNRKWTALHPGAKKMTEKWEKNRDVTMFFQKISLGDCKMWLEEFLMYWEQMLDPTKPPMV

SEQ ID NO: 16 - protein, 189 aa, Artificial Sequence
  Synthetic peptide ULBP2 alpha1-alpha2
AAEPHSLSYDITVIPKFRPGPRWCAVQGQVDEKTFLHYDCGNKTVTPVSPLGKKLNVTTAWKAQNPVLREVVDILTEQLRDIQLENYTPKEPLTLQARMSCEQKAEGHSSGSWQFSFDGQIFLLFDSEKRMWTTVHPGARKMKEKWENDKVVAMSFHYFSMGDCIGWLEDFLMGMDSTLEPSAGAPPMV

SEQ ID NO: 17 - protein, 187 aa, Artificial Sequence
  Synthetic peptide ULBP3 alpha1-alpha2
AAEPHSLWYNFTIIHLPRHGQQWCEVQSQVDQKNFLSYDCGSDKVLSMGHLEEQLYATDAWGKQLEMLREVGQRLRLELADTELEDFTPSGPLTLQVRMSCESEADGYIRGSWQFSFDGRKFLLFDSNNRKWTVVHAGARRMKEKWEKDSGLTTFFKMVSMRDCKSWLRDFLMHRKKRLEPTAPPMV

SEQ ID NO: 18 - protein, 187 aa, Artificial Sequence
  Synthetic peptide ULBP4 alpha1-alpha2
AAEPHSLCFNFTIKSLSRPGQPWCEAQVFLNKNLFLQYNSDNNMVKPLGLLGKKVYATSTWGELTQTLGEVGRDLRMLLCDIKPQIKTSDPSTLQVEMFCQREAERCTGASWQFATNGEKSLLFDAMNMTWTVINHEASKIKETWKKDRGLEKYFRKLSKGDCDHWLREFLGHWEAMPEPTVSPPMV

SEQ ID NO: 19 - protein, 189 aa, Artificial Sequence
  Synthetic peptide ULBP6 alpha1-alpha2
AAEPHSLCYDITVIPKFRPGPRWCAVQGQVDEKTFLHYDCGNKTVTPVSPLGKKLNVTTAWKAQNPVLREVVDILTEQLLDIQLENYTPKEPLTLQARMSCEQKAEGHSSGSWQFSIDGQTFLLFDSEKRMWTTVHPGARKMKEKWENDKDVAMSFHYISMGDCIGWLEDFLMGMDSTLEPSAGAPPMV

SEQ ID NO: 20 - protein, 161 aa, Artificial Sequence
  Synthetic peptide OMCP alpha1-alpha2
AAAEPHKLAFNFNLEINGSDTHSTVDVYLDDSQIITFDGKDIRPTIPFMIGDEIFLPFYKNVFSEFFSLFRRVPTSTPYEDLTYFYECDYTDNKSTFDQFYLYNGEEYTVKTQEATNKNMWLTTSEFRLKKWFDGEDCIMHLRSLVRKMEDSKRRTVPPMV

SEQ ID NO: 21 - protein, 580 aa, Artificial Sequence
  Synthetic peptide ULBP1-alpha3-iFv.2
MGLGPVFLLLAGIFPFAPPGAAAEPHCLCYDFIITPKSRPEPQWCEVQGLVDERPFLHYDCVNHKAKAFASLGKKVNVTKTWEEQTETLRDVVDFLKGQLLDIQVENLIPIEPLTLQARMSCEHEAHGHGRGSWQFLFNGQKFLLFDSNNRKWTALHPGAKKMTEKWEKNRDVTMFFQKISLGDCKMWLEEFLMYWEQMLDPTKPPMVQVTRSEASGGSGDRVTITCRASQDVSTAVAWYQQKPGKAPKLLIYSASFLYSGVPSRFSGSGSGTDFTLTISSLQPEDFATYYCQQSYTTPPTFGQGTKVEIKGGSSRSSSSGGGGSGGGGEVQLVESGGGLVQPGGSLRLSCAASGFTFTSTGISWVRQAPGKGLEWVGRIYPTNGSTNYADSVKGRFTISADTSKNTAYLQMNSLRAEDTAVYYCARTYGIYDLYVDYTEYVMDYWGQGTLVTVSSGGSSRSSSSGGGGSGGGGDIQMTQSPSSLSASGGSGQITVTCRASGFYPWNITLSWRQDGVSLSHDTQQWGDVLPDGQGTYQTWVATRISQGEEQRFTCYMEHSGQHSTHPVPSGKGSHHHHHH

SEQ ID NO: 22 - protein, 582 aa, Artificial Sequence
  Synthetic peptide ULBP2-alpha3-iFv.2
MGLGPVFLLLAGIFPFAPPGAAAEPHSLCYDITVIPKFRPGPRWCAVQGQVDEKTFLHYDCGNKTVTPVSPLGKKLNVTTAWKAQNPVLREVVDILTEQLRDIQLENYTPKEPLTLQARMSCEQKAEGHSSGSWQFSFDGQIFLLFDSEKRMWTTVHPGARKMKEKWENDKVVAMSFHYFSMGDCIGWLEDFLMGMDSTLEPSAGAPPMVQVTRSEASGGSGDRVTITCRASQDVSTAVAWYQQKPGKAPKLLIYSASFLYSGVPSRFSGSGSGTDFTLTISSLQPEDFATYYCQQSYTTPPTFGQGTKVEIKGGSSRSSSSGGGGSGGGGEVQLVESGGGLVQPGGSLRLSCAASGFTFTSTGISWVRQAPGKGLEWVGRIYPTNGSTNYADSVKGRFTISADTSKNTAYLQMNSLRAEDTAVYYCARTYGIYDLYVDYTEYVMDYWGQGTLVTVSSGGSSRSSSSGGGGSGGGGDIQMTQSPSSLSASGGSGQITVTCRASGFYPWNITLSWRQDGVSLSHDTQQWGDVLPDGQGTYQTWVATRISQGEEQRFTCYMEHSGQHSTHPVPSGKGSHHHHHH

SEQ ID NO: 23 - protein, 580 aa, Artificial Sequence
  Synthetic peptide ULBP3-alpha3-iFv.2
MGLGPVFLLLAGIFPFAPPGAAAEPHSLWYNFTIIHLPRHGQQWCEVQSQVDQKNFLSYDCGSDKVLSMGHLEEQLYATDAWGKQLEMLREVGQRLRLELADTELEDFTPSGPLTLQVRMSCECEADGYIRGSWQFSFDGRKFLLFDSNNRKWTVVHAGARRMKEKWEKDSGLTTFFKMVSMRDCKSWLRDFLMHRKKRLEPTAPPMVQVTRSEASGGSGDRVTITCRASQDVSTAVAWYQQKPGKAPKLLIYSASFLYSGVPSRFSGSGSGTDFTLTISSLQPEDFATYYCQQSYTTPPTFGQGTKVEIKGGSSRSSSSGGGGSGGGGEVQLVESGGGLVQPGGSLRLSCAASGFTFTSTGISWVRQAPGKGLEWVGRIYPTNGSTNYADSVKGRFTISADTSKNTAYLQMNSLRAEDTAVYYCARTYGIYDLYVDYTEYVMDYWGQGTLVTVSSGGSSRSSSSGGGGSGGGGDIQMTQSPSSLSASGGSGQITVTCRASGFYPWNITLSWRQDGVSLSHDTQQWGDVLPDGQGTYQTWVATRISQGEEQRFTCYMEHSGQHSTHPVPSGKGSHHHHHH

SEQ ID NO: 24 - protein, 580 aa, Artificial Sequence
  Synthetic peptide ULBP4-alpha3-iFv.2
MGLGPVFLLLAGIFPFAPPGAAAEPHSLCFNFTIKSLSRPGQPWCEAQVFLNKNLFLQYNSDNNMVKPLGLLGKKVYATSTWGELTQTLGEVGRDLRMLLCDIKPQIKTSDPSTLQVEMFCQREAERCTGASWQFATNGEKSLLFDAMNMTWTVINHEASKIKETWKKDRGLEKYFRKLSKGDCDHWLREFLGHWEAMPEPTVSPPMVQVTRSEASGGSGDRVTITCRASQDVSTAVAWYQQKPGKAPKLLIYSASFLYSGVPSRFSGSGSGTDFTLTISSLQPEDFATYYCQQSYTTPPTFGQGTKVEIKGGSSRSSSSGGGGSGGGGEVQLVESGGGLVQPGGSLRLSCAASGFTFTSTGISWVRQAPGKGLEWVGRIYPTNGSTNYADSVKGRFTISADTSKNTAYLQMNSLRAEDTAVYYCARTYGIYDLYVDYTEYVMDYWGQGTLVTVSSGGSSRSSSSGGGGSGGGGDIQMTQSPSSLSASGGSGQITVTCRASGFYPWNITLSWRQDGVSLSHDTQQWGDVLPDGQGTYQTWVATRISQGEEQRFTCYMEHSGQHSTHPVPSGKGSHHHHHH

SEQ ID NO: 25 - protein, 582 aa, Artificial Sequence
  Synthetic peptide ULBP6-alpha3-iFv.2
MGLGPVFLLLAGIFPFAPPGAAAEPHSLCYDITVIPKFRPGPRWCAVQGQVDEKTFLHYDCGNKTVTPVSPLGKKLNVTTAWKAQNPVLREVVDILTEQLLDIQLENYTPKEPLTLQARMSCEQKAEGHSSGSWQFSIDGQTFLLFDSEKRMWTTVHPGARKMKEKWENDKDVAMSFHYISMGDCIGWLEDFLMGMDSTLEPSAGAPPMVQVTRSEASGGSGDRVTITCRASQDVSTAVAWYQQKPGKAPKLLIYSASFLYSGVPSRFSGSGSGTDFTLTISSLQPEDFATYYCQQSYTTPPTFGQGTKVEIKGGSSRSSSSGGGGSGGGGEVQLVESGGGLVQPGGSLRLSCAASGFTFTSTGISWVRQAPGKGLEWVGRIYPTNGSTNYADSVKGRFTISADTSKNTAYLQMNSLRAEDTAVYYCARTYGIYDLYVDYTEYVMDYWGQGTLVTVSSGGSSRSSSSGGGGSGGGGDIQMTQSPSSLSASGGSGQITVTCRASGFYPWNITLSWRQDGVSLSHDTQQWGDVLPDGQGTYQTWVATRISQGEEQRFTCYMEHSGQHSTHPVPSGKGSHHHHHH

SEQ ID NO: 26 - protein, 553 aa, Artificial Sequence
  Synthetic peptide OMCP-alpha3-iFv.2
MGLGPVFLLLAGIFPFAPPGAAAEPHKLAFNFNLEINGSDTHSTVDVYLDDSQIITFDGKDIRPTIPFMIGDEIFLPFYKNVFSEFFSLFRRVPTSTPYEDLTYFYECDYTDNKSTFDQFYLYNGEEYTVKTQEATNKNMWLTTSEFRLKKWFDGEDCIMHLRSLVRKMEDSKRRTVPPMVQVTRSEASGGSGDRVTITCRASQDVSTAVAWYQQKPGKAPKLLIYSASFLYSGVPSRFSGSGSGTDFTLTISSLQPEDFATYYCQQSYTTPPTFGQGTKVEIKGGSSRSSSSGGGGSGGGGEVQLVESGGGLVQPGGSLRLSCAASGFTFTSTGISWVRQAPGKGLEWVGRIYPTNGSTNYADSVKGRFTISADTSKNTAYLQMNSLRAEDTAVYYCARTYGIYDLYVDYTEYVMDYWGQGTLVTVSSGGSSRSSSSGGGGSGGGGDIQMTQSPSSLSASGGSGQITVTCRASGFYPWNITLSWRQDGVSLSHDTQQWGDVLPDGQGTYQTWVATRISQGEEQRFTCYMEHSGQHSTHPVPSGKGSHHHHHH

SEQ ID NO: 27 - DNA, 507 bp, Artificial Sequence
  Synthetic polynucleotide, encoding alpha1-alpha2 variant 15
gctgctgagccacacagtctccgctacaaccttacggtgttgagctgggacggctctgtccagagtggctttctgactgaggtacatctcgatggtcagcccttcctccgatgcgacagacaaaagtgcagggccaagccacagggccaatgggccgaagatgtacttggcaataagacttgggacagagaaaccagagatctgactggctggggtaaggacttacgcatgactctcgcacacattaaagaccagaaggaaggtcttcattcgctccaggaaattagagtctgtgaaatccatgaagacaacagcacaagaagttcccaacatttctactacgacggcgagctgttcttatcacagaatttagagaccaacgagtggacaatgccccaaagctcgagggcccagaccctcgctatgaatgtgaggaatttccttaaggaggacgctatggaaactgacacccactaccatgcgatgcgcgccgattgcctgcaggaa

SEQ ID NO: 28 - DNA, 507 bp, Artificial Sequence
  Synthetic polynucleotide, encoding alpha1-alpha2 variant 16
gctgctgagccacacagtctccgctacaaccttacggtgttgagctgggacggctctgtccagagtggctttctgactgaggtacatctcgatggtcagcccttcctccgatgcgacagacaaaagtgcagggccaagccacagggccaatgggccgaagatgtacttggcaataagacttgggacagagaaaccagagatctgactggctggggtaaggacttacgcatgactctcgcacacattaaagaccagaaggaaggtcttcattcgctccaggaaattagagtctgtgaaatccatgaagacaacagcacaagaagttcccaacatttctactacgacggcgagctgttcttatcacagaatttagagaccctcgagtggacaatgccccaaagctcgagggcccagaccctcgctatgaatgtgaggaatttccttaaggaggacgctatggaaactgacacccactaccatgcgatgcgcgccgattgcctgcaggaa

SEQ ID NO: 29 - DNA, 507 bp, Artificial Sequence
  Synthetic polynucleotide, encoding alpha1-alpha2 variant 17
gctgctgagccacacagtctccgctacaaccttacggtgttgagctgggacggctctgtccagagtggctttctgactgaggtacatctcgatggtcagcccttcctccgatgcgacagacaaaagtgcagggccaagccacagggccaatgggccgaagatgtacttggcaataagacttgggacagagaaaccagagatctgactctctggggtaaggacttacgcatgactctcgcacacattaaagaccagaaggaaggtcttcattcgctccaggaaattagagtctgtgaaatccatgaagacaacagcacaagaagttcccaacatttctactacgacggcgagctgttcttatcacagaatttagagaccctcgagtggacaatgccccaaagctcgagggcccagaccctcgctatgaatgtgaggaatttccttaaggaggacgctatggaaactgacacccactaccatgcgatgcgcgccgattgcctgcaggaa

SEQ ID NO: 30 - DNA, 507 bp, Artificial Sequence
  Synthetic polynucleotide, encoding alpha1-alpha2 variant 18
gctgctgagccacacagtctccgctacaaccttacggtgttgagctgggacggctctgtccagcccggctttctgactgaggtacatctcgatggtcagcccttcctccgatgcgacagacaaaagtgcagggccaagccacagggccaatgggccgaagatgtacttggcaataagacttgggacagagaaaccagagatctgactctctggggtaaggacttacgcatgactctcgcacacattaaagaccagaaggaaggtcttcattcgctccaggaaattagagtctgtgaaatccatgaagacaacagcacaagaagttcccaacatttctactacgacggcgagctgttcttatcacagaatttagagaccctcgagtggacaatgccccaaagctcgagggcccagaccctcgctatgaatgtgaggaatttccttaaggaggacgctatggaaactgacacccactaccatgcgatgcgcgccgattgcctgcaggaa

SEQ ID NO: 31 - protein, 558 aa, Artificial Sequence
  Synthetic peptide MICA alpha1-alpha2 variant 15
EPHSLRYNLTVLSWDGSVQSGFLTEVHLDGQPFLRCDRQKCRAKPQGQWAEDVLGNKTWDRETRDLTGWGKDLRMTLAHIKDQKEGLHSLQEIRVCEIHEDNSTRSSQHFYYDGELFLSQNLETNEWTMPQSSRAQTLAMNVRNFLKEDAMETDTHYHAMRADCLQELRRYLKSGVVLRRTVPPMVQVTRSEASGGSGDRVTITCRASQDVSTAVAWYQQKPGKAPKLLIYSASFLYSGVPSRFSGSGSGTDFTLTISSLQPEDFATYYCQQSYTTPPTFGQGTKVEIKGGSSRSSSSGGGGSGGGGEVQLVESGGGLVQPGGSLRLSCAASGFTFTSTGISWVRQAPGKGLEWVGRIYPTNGSTNYADSVKGRFTISADTSKNTAYLQMNSLRAEDTAVYYCARTYGIYDLYVDYTEYVMDYWGQGTLVTVSSGGSSRSSSSGGGGSGGGGDIQMTQSPSSLSASGGSGQITVTCRASGFYPWNITLSWRQDGVSLSHDTQQWGDVLPDGQGTYQTWVATRISQGEEQRFTCYMEHSGQHSTHPVPSGKGSHHHHHH

SEQ ID NO: 32 - protein, 558 aa, Artificial Sequence
  Synthetic peptide MICA alpha1-alpha2 variant 16
EPHSLRYNLTVLSWDGSVQSGFLTEVHLDGQPFLRCDRQKCRAKPQGQWAEDVLGNKTWDRETRDLTGWGKDLRMTLAHIKDQKEGLHSLQEIRVCEIHEDNSTRSSQHFYYDGELFLSQNLETLEWTMPQSSRAQTLAMNVRNFLKEDAMETDTHYHAMRADCLQELRRYLKSGVVLRRTVPPMVQVTRSEASGGSGDRVTITCRASQDVSTAVAWYQQKPGKAPKLLIYSASFLYSGVPSRFSGSGSGTDFTLTISSLQPEDFATYYCQQSYTTPPTFGQGTKVEIKGGSSRSSSSGGGGSGGGGEVQLVESGGGLVQPGGSLRLSCAASGFTFTSTGISWVRQAPGKGLEWVGRIYPTNGSTNYADSVKGRFTISADTSKNTAYLQMNSLRAEDTAVYYCARTYGIYDLYVDYTEYVMDYWGQGTLVTVSSGGSSRSSSSGGGGSGGGGDIQMTQSPSSLSASGGSGQITVTCRASGFYPWNITLSWRQDGVSLSHDTQQWGDVLPDGQGTYQTWVATRISQGEEQRFTCYMEHSGQHSTHPVPSGKGSHHHHHH

SEQ ID NO: 33 - protein, 558 aa, Artificial Sequence
  Synthetic peptide MICA alpha1-alpha2 variant 17
EPHSLRYNLTVLSWDGSVQSGFLTEVHLDGQPFLRCDRQKCRAKPQGQWAEDVLGNKTWDRETRDLTLWGKDLRMTLAHIKDQKEGLHSLQEIRVCEIHEDNSTRSSQHFYYDGELFLSQNLETLEWTMPQSSRAQTLAMNVRNFLKEDAMETDTHYHAMRADCLQELRRYLKSGVVLRRTVPPMVQVTRSEASGGSGDRVTITCRASQDVSTAVAWYQQKPGKAPKLLIYSASFLYSGVPSRFSGSGSGTDFTLTISSLQPEDFATYYCQQSYTTPPTFGQGTKVEIKGGSSRSSSSGGGGSGGGGEVQLVESGGGLVQPGGSLRLSCAASGFTFTSTGISWVRQAPGKGLEWVGRIYPTNGSTNYADSVKGRFTISADTSKNTAYLQMNSLRAEDTAVYYCARTYGIYDLYVDYTEYVMDYWGQGTLVTVSSGGSSRSSSSGGGGSGGGGDIQMTQSPSSLSASGGSGQITVTCRASGFYPWNITLSWRQDGVSLSHDTQQWGDVLPDGQGTYQTWVATRISQGEEQRFTCYMEHSGQHSTHPVPSGKGSHHHHHH

SEQ ID NO: 34 - protein, 558 aa, Artificial Sequence
  Synthetic peptide MICA alpha1-alpha2 variant 18
EPHSLRYNLTVLSWDGSVQPGFLTEVHLDGQPFLRCDRQKCRAKPQGQWAEDVLGNKTWDRETRDLTLWGKDLRMTLAHIKDQKEGLHSLQEIRVCEIHEDNSTRSSQHFYYDGELFLSQNLETLEWTMPQSSRAQTLAMNVRNFLKEDAMETDTHYHAMRADCLQELRRYLKSGVVLRRTVPPMVQVTRSEASGGSGDRVTITCRASQDVSTAVAWYQQKPGKAPKLLIYSASFLYSGVPSRFSGSGSGTDFTLTISSLQPEDFATYYCQQSYTTPPTFGQGTKVEIKGGSSRSSSSGGGGSGGGGEVQLVESGGGLVQPGGSLRLSCAASGFTFTSTGISWVRQAPGKGLEWVGRIYPTNGSTNYADSVKGRFTISADTSKNTAYLQMNSLRAEDTAVYYCARTYGIYDLYVDYTEYVMDYWGQGTLVTVSSGGSSRSSSSGGGGSGGGGDIQMTQSPSSLSASGGSGQITVTCRASGFYPWNITLSWRQDGVSLSHDTQQWGDVLPDGQGTYQTWVATRISQGEEQRFTCYMEHSGQHSTHPVPSGKGSHHHHHH

SEQ ID NO: 35 - protein, 558 aa, Artificial Sequence
  Synthetic peptide MICA-WED
EPHSLRYNLTVLSWDGSVQSGFLTEVHLDGQPFLRCDRQKCRAKPQGQWAEDVLGNKTWDRETRDLTGWGKDLRMTLAHIKDQKEGLHSLQEIRVCEIHEDNSTRSSQHFYYDGELFLSQNLETKEWTMPQSSRAQTLAMNVRNFLKEDAMETDTHYHAMHADCLQELRRYLKSGVVLRRTVPPMVQVTRSEASGGSGDRVTITCRASQDVSTAVAWYQQKPGKAPKLLIYSASFLYSGVPSRFSGSGSGTDFTLTISSLQPEDFATYYCQQSYTTPPTFGQGTKVEIKGGSSRSSSSGGGGSGGGGEVQLVESGGGLVQPGGSLRLSCAASGFTFTSTGISWVRQAPGKGLEWVGRIYPTNGSTNYADSVKGRFTISADTSKNTAYLQMNSLRAEDTAVYYCARTYGIYDLYVDYTEYVMDYWGQGTLVTVSSGGSSRSSSSGGGGSGGGGDIQMTQSPSSLSASGGSGQITVTCRASGFYPWNITLSWRQDGVSLSHDTQQWGDVLPDGQGTYQTWVATRISQGEEQRFTCYMEHSGQHSTHPVPSGKGSHHHHHH

SEQ ID NO: 36 - protein, 274 aa, Artificial Sequence
  Synthetic peptide MICA
EPHSLRYNLTVLSWDGSVQSGFLTEVHLDGQPFLRCDRQKCRAKPQGQWAEDVLGNKTWDRETRDLTGNGKDLRMTLAHIKDQKEGLHSLQEIRVCEIHEDNSTRSSQHFYYDGELFLSQNLETEEWTMPQSSRAQTLAMNVRNFLKEDAMKTKTLYHAMHADCLQELRRYLKSGVVLRRTVPPMVNVTRSEASEGNITVTCRASGFYPWNITLSWRQDGVSLSHDTQQWGDVLPDGNGTYQTWVATRICQGEEQRFTCYMEHSGNHSTHPVPS

SEQ ID NO: 37 - protein, 274 aa, Artificial Sequence
  Synthetic peptide MICA
EPHSLRYNLTVLSWDGSVQSGFLAEVHLDGQPFLRCDRQKCRAKPQGQWAEDVLGNKTWDRETRDLTGNGKDLRMTLAHIKDQKEGLHSLQEIRVCEIHEDNSTRSSQHFYYDGELFLSQNLETEEWTMPQSSRAQTLAMNIRNFLKEDAMKTKTHYHAMHADCLQELRRYLKSGVVLRRTVPPMVNVTRSEASEGNITVTCRASGFYPWNITLSWRQDGVSLSHDTQQWGDVLPDGNGTYQTWVATRICQGEEQRFTCYMEHSGNHSTHPVPS

SEQ ID NO: 38 - protein, 274 aa, Artificial Sequence
  Synthetic peptide MICA
EPHSLPYNLTVLSWDGSVQSGFLAEVHLDGQPFLRYDRQKCRAKPQGQWAEDVLGNKTWDRETRDLTGNGKDLRMTLAHIKDQKEGLHSLQEIRVCEIHEDNSTRSSQHFYYDGELFLSQNLETEEWTMPQSSRAQTLAMNVRNFLKEDAMKTKTHYHAMHADCLQELRRYLKSGVVLRRTVPPMVNVTRSEASEGNITVTCRASGFYPWNITLSWRQDGVSLSHDTQQWGDVLPDGNGTYQTWVATRICQGEEQRFTCYMEHSGNHSTHPVPS

SEQ ID NO: 39 - protein, 274 aa, Artificial Sequence
  Synthetic peptide MICA
EPHSLRYNLTVLSWDGSVQSGFLAEVHLDGQPFLRYDRQKCRAKPQGQWAEDVLGNKTWDRETRDLTGNGKDLRMTLAHIKDQKEGLHSLQEIRVCEIHEDNSTRSSQHFYYDGELFLSQNLETEEWTVPQSSRAQTLAMNVRNFLKEDAMKTKTHYHAMHADCLQELRRYLESGVVLRRTVPPMVNVTRSEASEGNITVTCRASSFYPRNITLTWRQDGVSLSHDTQQWGDVLPDGNGTYQTWVATRICQGEEQRFTCYMEHSGNHSTHPVPS

SEQ ID NO: 40 - protein, 274 aa, Artificial Sequence
  Synthetic peptide MICA
EPHSLRYNLTVLSWDGSVQSGFLTEVHLDGQPFLRCDRQKCRAKPQGQWAEDVLGNKTWDRETRDLTGNGKDLRMTLAHIKDQKEGLHSLQEIRVCEIHEDNSTRSSQHFYYDGELFLSQNLETEEWTMPQSSRAQTLAMNVRNFLKEDAMKTKTHYHAMHADCLQELRRYLKSGVVLRRTVPPMVNVTRSEASEGNITVTCRASGFYPWNITLSWRQDGVSLSHDTQQWGDVLPDGNGTYQTWVATRICQGEEQRFTCYMEHSGNHSTHPVPS

SEQ ID NO: 41 - protein, 274 aa, Artificial Sequence
  Synthetic peptide MICA
EPHSLRYNLTVLSWDGSVQSGFLAEVHLDGQPFLRCDRQKCRAKPQGQWAEDVLGNKTWDRETRDLTGNGKDLRMTLAHIKDQKEGLHSLQEIRVCEIHEDNSTRSSQHFYYDGELFLSQNLETEEWTMPQSSRAQTLAMNVRNFLKEDAMKTKTHYHAMHADCLQELRRYLKSGVVLRRTVPPMVNVTRSEASEGNITVTCRASGFYPWNITLSWRQDGVSLSHDTQQWGDVLPDGNGTYQTWVATRICQGEEQRFTCYMEHSGNHSTHPVPS

SEQ ID NO: 42 - protein, 276 aa, Artificial Sequence
  Synthetic peptide MICA
EPHSLRYNLTVLSWDGSVQSGFLTEVHLDGQPFLRCDRQKCRAKPQGQWAEDVLGNKTWDRETRDLTGNGKDLRMTLAHIKDQKEGLHSLQEIRVCEIHEDNSTRSSQHFYYDGELFLSQNLETKEWTMPQSSRAQTLAMNVRNFLKEDAMKTKTHYHAMHADCLQELRRYLKSGVVLRRTVPPMVNVTRSEASEGNITVTCRASGFYPWNITLSWRQDGVSLSHDTQQWGDVLPDGNGTYQTWVATRICQGEEQRFTCYMEHSGNHSTHPVPSGK

SEQ ID NO: 43 - protein, 306 aa, Artificial Sequence
  Synthetic peptide MICB
EPHSLRYNLMVLSQDGSVQSGFLAEGHLDGQPFLRYDRQKRRAKPQGQWAEDVLGAKTWDTETEDLTENGQDLRRTLTHIKDQKGGLHSLQEIRVCEIHEDSSTRGSRHFYYDGELFLSQNLETQESTVPQSSRAQTLAMNVTNFWKEDAMKTKTHYRAMQADCLQKLQLPPMVNVICSEVSEGNITVTCRASSFYPRNITLTWRQDGVSLSHNTQQWGDVLPDGNGTYQTWVATRIRQGEEQRFTCYMEHSGNHGTHPVPSGKALVLQSQRTDFPYVSAAMPCFVIIIILCVPCCKKKTSAAEGP

SEQ ID NO: 44 - protein, 318 aa, Artificial Sequence
  Synthetic peptide MICB
EPHSLRYNLMVLSQDGSVQSGFLAEGHLDGQPFLRYDRQKRRAKPQGQWAEDVLGAETWDTETEDLTENGQDLRRTLTHIKDQKGGLHSLQEIRVCEMHEDSSTRGSRHFYYNGELFLSQNLETQESTVPQSSRAQTLAMNVTNFWKEDAMKTKTHYRAMQADCLQKLQRYLKSGVAIRRTVPPMVNVTCSEVSEGNITVTCRASSFYPRNITLTWRQDGVSLSHNTQQWGDVLPDGNGTYQTWVATRIRQGEEQRFTCYMEHSGNHGTHPVPSGKALVLQSQRTDFPYVSAAMPCFVIIIILCVPCCKKKTSAAEGP

SEQ ID NO: 45 - protein, 318 aa, Artificial Sequence
  Synthetic peptide MICB
EPHSLRYNLMVLSQDGSVQSGFLAEGHLDGQPFLRYDRQKRRAKPQGQWAEDVLGAKTWDTETEDLTENGQDLRRTLTHIKDQKGGLHSLQEIRVCEIHEDSSTRGSRHFYYDGELFLSQNLETQESTVPQSSRAQTLAMNVTNFWKEDAMKTKTHYRAMQADCLQKLQRYLKSGVAIRRTVPPMVNVICSEVSEGNITVTCRASSFYPRNITLTWRQDGVSLSHNTQQWGDVLPDGNGTYQTWVATRIRQGEEQRFTCYMEHSGNHGTHPVPSGKALVLQSQRTDFPYVSAAMPCFVIIIILCVPCCKKKTSAAEGP

SEQ ID NO: 46 - protein, 318 aa, Artificial Sequence
  Synthetic peptide MICB
EPHSLRYNLMVLSQDGSVQSGFLAEGHLDGQPFLRYDRQKRRAKPQGQWAENVLGAKTWDTETEDLTENGQDLRRTLTHIKDQKGGLHSLQEIRVCEIHEDSSTRGSRHFYYDGELFLSQNLETQESTVPQSSRAQTLAMNVTNFWKEDAMKTKTHYRAMQADCLQKLQRYLKSGVAIRRTVPPMVNVTCSEVSEGNITVTCRASSFYPRNITLTWRQDGVSLSHNTQQWGDVLPDGNGTYQTWVATRIRQGEEQRFTCYMEHSGNHGTHPVPSGKALVLQSQRTDFPYVSAAMPCFVIIIILCVPCCKKKTSAAEGP

SEQ ID NO: 47 - protein, 318 aa, Artificial Sequence
  Synthetic peptide MICB
EPHSLRYNLMVLSQDGSVQSGFLAEGHLDGQPFLRYDRQKRRAKPQGQWAEDVLGAETWDTETEDLTENGQDLRRTLTHIKDQKGGLHSLQEIRVCEIHEDSSTRGSRHFYYNGELFLSQNLETQESTVPQSSRAQTLAMNVTNFWKEDAMKTKTHYRAMQADCLQKLQRYLKSGVAIRRTVPPMVNVTCSEVSEGNITVTCRASSFYPRNITLTWRQDGVSLSHNTQQWGDVLPDGNGTYQTWVATRIRQGEEQKFTCYMEHSGNHGTHPVPSGKALVLQSQRTDFPYVSAAMPCFVIIIILCVPCCKKKTSAAEGP

SEQ ID NO: 48 - protein, 318 aa, Artificial Sequence
  Synthetic peptide MICB
EPHSLRYNLMVLSQDGSVQSGFLAEGHLDGQPFLRYDRQKRRAKPQGQWAEDVLGAETWDTETEDLTENGQDLRRTLTHIKDQKGGLHSLQEIRVCEIHEDSSTRGSRHFYYNGELFLSQNLETQESTVPQSSRAQTLAMNVTNFWKEDAMKTKTHYRAMQADCLQKLQRYLKSGVAIRRTVPPMVNVTCSEVSEGNITVTCRASSFYPRNITLTWRQDGVSLSHNTQQWGDVLPDGNGTYQTWVATRIRQGEEQRFTCYMEHSGNHGTHPVPSGKALVLQSQRTDFPYVSAAMPCFVIIIILCVPCCKKKTSAAEGP

SEQ ID NO: 49 - protein, 244 aa, Artificial Sequence
  Synthetic peptide ULBP-1 (ACCESSION NO Q9BZM6)
MAAAASPAFLLCLPLLHLLSGWSRAGWVDTHCLCYDFIITPKSRPEPQWCEVQGLVDERPFLHYDCVNHKAKAFASLGKKVNVTKTWEEQTETLRDVVDFLKGQLLDIQVENLIPIEPLTLQARMSCEHEAHGHGRGSWQFLFNGQKFLLFDSNNRKWTALHPGAKKMTEKWEKNRDVTMFFQKISLGDCKMWLEEFLMYWEQMLDPTKPPSLAPGTTQPKAMATTLSPWSLLIIFLCFILAGR

SEQ ID NO: 50 - protein, 246 aa, Artificial Sequence
  Synthetic peptide ULBP-2 (ACCESSION NO Q9BZM5)
MAAAAATKILLCLPLLLLLSGWSRAGRADPHSLCYDITVIPKFRPGPRWCAVQGQVDEKTFLHYDCGNKTVTPVSPLGKKLNVTTAWKAQNPVLREVVDILTEQLRDIQLENYTPKEPLTLQARMSCEQKAEGHSSGSWQFSFDGQIFLLFDSEKRMWTTVHPGARKMKEKWENDKVVAMSFHYFSMGDCIGWLEDFLMGMDSTLEPSAGAPLAMSSGTTQLRATATTLILCCLLIILPCFILPGI

SEQ ID NO: 51 - protein, 244 aa, Artificial Sequence
  Synthetic peptide ULBP-3 (ACCESSION NO NP_078794)
MAAAASPAILPRLAILPYLLFDWSGTGRADAHSLWYNFTIIHLPRHGQQWCEVQSQVDQKNFLSYDCGSDKVLSMGHLEEQLYATDAWGKQLEMLREVGQRLRLELADTELEDFTPSGPLTLQVRMSCECEADGYIRGSWQFSFDGRKFLLFDSNNRKWTVVHAGARRMKEKWEKDSGLTTFFKMVSMRDCKSWLRDFLMHRKKRLEPTAPPTMAPGLAQPKAIATTLSPWSFLIILCFILPGI

SEQ ID NO: 52 - protein, 263 aa, Artificial Sequence
  Synthetic peptide ULBP-4/RAET1E (ACCESSION NO Q8TD07)
MRRISLTSSPVRLLLFLLLLLIALEIMVGGHSLCFNFTIKSLSRPGQPWCEAQVFLNKNLFLQYNSDNNMVKPLGLLGKKVYATSTWGELTQTLGEVGRDLRMLLCDIKPQIKTSDPSTLQVEMFCQREAERCTGASWQFATNGEKSLLFDAMNMTWTVINHEASKIKETWKKDRGLEKYFRKLSKGDCDHWLREFLGHWEAMPEPTVSPVNASDIHWSSSSLPDRWIILGAFILLVLMGIVLICVWWQNGEWQAGLWPLRTS

SEQ ID NO: 53 - protein, 332 aa, Artificial Sequence
  Synthetic peptide ULBP-5 (ACCESSION NO Q6H3X3)
MAAAASPAFLLRLPLLLLLSSWCRTGLADPHSLCYDITVPKFRPGPRWCAVQGQVDEKTFLHYDCGSKTVTPVSPLGKKLNVTTAWKAQNPVLREVVDLTEQLLDIQLENYIPKEPLTLQARMSCEQKAEGHGSGSWQLSFDGQIFLLFDSENRMWTTVHPGARKMKEKWENDKDMTMSFHYISMGDCTGWLEDFLMGMDSTLEPSAGAPPTMSSGTAQPRATATTLILCCLLIMCLLICSRHSLTQSHGHHPQSLQPPPHPPLLHPTWLLRRVLWSDSYQIAKRPLSGGHVTRVTLPIIGDDSHSLPCPLALYTINNGAARYSEPLQVSIS

SEQ ID NO: 54 - protein, 246 aa, Artificial Sequence
  Synthetic peptide ULBP-6 (ACCESSION NO NP_570970)
MAAAAIPALLLCLPLLFLLFGWSRARRDDPHSLCYDITVIPKFRPGPRWCAVQGQVDEKTFLHYDCGNKTVTPVSPLGKKLNVTMAWKAQNPVLREVVDILTEQLLDIQLENYTPKEPLTLQARMSCEQKAEGHSSGSWQFSIDGQTFLLFDSEKRMWTTVHPGARKMKEKWENDKDVAMSFHYISMGDCIGWLEDFLMGMDSTLEPSAGAPLAMSSGTTQLRATATTLILCCLLIILPCFILPGI

SEQ ID NO: 55 - protein, 182 aa, Artificial Sequence
  Synthetic peptide MICwed alpha1-alpha2
EPHSLRYNLTVLSWDGSVQSGFLTEVHLDGQPFLRCDRQKCRAKPQGQWAEDVLGNKTWDRETRDLTGWGKDLRMTLAHIKDQKEGLHSLQEIRVCEIHEDNSTRSSQHFYYDGELFLSQNLETKEWTMPQSSRAQTLAMNVRNFLKEDAMETDTHYHAMHADCLQELRRYLKSGVVLRRTV

SEQ ID NO: 56 - protein, 182 aa, Artificial Sequence
  Synthetic peptide DSM20 alpha1-alpha2
EPHSLRYNLTVLSWDGSVQSGFLTEVHLDGQPFLRCDRQKCRAKPQGQWAEDVLGNKTWDRETRDLTAWGKDLRMTLAHIKDQKEGLHSLQEIRVCEIHEDNSTRSSQHFYYDGELFLSQNLETLEWTMPQSSRAQTLAMNVRNFLKEDAMQTDTHYRAMHADCLFELRRYLKSGVVLRRTV

SEQ ID NO: 57 - protein, 182 aa, Artificial Sequence
  Synthetic peptide DSM25 alpha1-alpha2
EPHSLRYNLTVLSWDGSVQSGFLTEVHLDGQPFLRCDRQKCRAKPQGQWAEDVLGNKTWDRETRDLTGWGKDLRMTLAHIKDQKEGLHSLQEIRVCEIHEDNSTRSSQHFYYDGELFLSQNLETLEWTMPQSSRAQTLAMNVRNFLKEDAMETDTHYHAMRADCLSELRRYLKSGVVLRRTV

SEQ ID NO: 58 - protein, 182 aa, Artificial Sequence
  Synthetic peptide DSM27 alpha1-alpha2
EPHSLRYNLTVLSWDGSVQSGFLTEVHLDGQPFLRCDRQKCRAKPQGQWAEDVLGNKTWDRETRDLTGWGKDLRMTLAHIKDQKEGLHSLQEIRVCEIHEDNSTRSSQHFYYDGELFLSQNLETLEWTMPQSSRAQTLAMNVRNFLKEDAMKTKTHYHAMRADCLSELRRYLKSGVVLRRTV

SEQ ID NO: 59 - protein, 182 aa, Artificial Sequence
  Synthetic peptide DSM28 alpha1-alpha2
EPHSLRYNLTVLSWDGSVQSGFLTEVHLDGQPFLRCDRQKCRAKPQGQWAEDVLGNKTWDRETRDLTGNGKDLRMTLAHIKDQKEGLHSLQEIRVCEIHEDNSTRSSQHFYYDGELFLSQNLETLEWTMPQSSRAQTLAMNVRNFLKEDAMKTKTHYHAMRADCLSELRRYLKSGVVLRRTV

SEQ ID NO: 60 - protein, 182 aa, Artificial Sequence
  Synthetic peptide DSM42 alpha1-alpha2
EPHSLRYNLTVLSWDGSVQSGFLTEVHLDGQPFLRCDRQKCRAKPQGQWAEDVLGNKTWDRETRDLTGWGKDLRMTLAHIKDQKEGLHSLQEIRVCEIHEDNSTRSSQHFYYDGELFLSQNLETLEWTMPQSSRAQTLAMNVRNFLKEDAMETDTHYHAMRADCLQELRRYLKSGVVLRRTV

SEQ ID NO: 61 - protein, 182 aa, Artificial Sequence
  Synthetic peptide DSM48 alpha1-alpha2
EPHSLRYNLTVLSWDGSVQSGFLTEVHLDGQPFLRCDRQKCRAKPQGQWAEDVLGNKTWDRETRDLTGWGKDLRMTLAHIKDQKEGLHSLQEIRVCEIHEDNSTRSSQHFYYDGELFLSQNLETLEWTMPQSSRAQTLAMNVRNFLKEDAMATDTHYIAMRADCLAELRRYLKSGVVLRRTV

SEQ ID NO: 62 - protein, 182 aa, Artificial Sequence
  Synthetic peptide DSM49 alpha1-alpha2
EPHSLRYNLTVLSWDGSVQTGFLTEVHLDGQPFLRCDRQKCRAKPQGQWAEDVLGNKTWDRETRDLTQWGKDLRMTLAHIKDQKEGLHSLQEIRVCEIHEDNSTRSSQHFYYDGELFLSQNLETKEWTMPQSSRAQTLAMNVRNFLKEDAMFTDTHYRAMTADCLTELRRYLKSGVVLRRTV

SEQ ID NO: 63 - DNA, 29 bp, Artificial Sequence
  Synthetic oligonucleotide primer
atctataatgctgagccccacagtcttcg

SEQ ID NO: 64 - DNA, 27 bp, Artificial Sequence
  Synthetic oligonucleotide primer
cttgctcttcagatatcgccgtagttc

SEQ ID NO: 65 - DNA, 7556 bp, Artificial Sequence
  Synthetic DNA construct expressing wt a1a2 domain-Fv
ggagagaccacacccaagctgtctagagccgccacgatggggctgggcccggtcttcctgcttctggctggcatcttcccttttgcacctccgggagctgctgctgagccccacagtcttcgttataacctcacggtgctgtcctgggatggatctgtgcagtcagggtttctcactgaggtacatctggatggtcagcccttcctgcgctgtgacaggcagaaatgcagggcaaagccccagggacagtgggcagaagatgtcctgggaaataagacatgggacagagagaccagagacttgacagggaatggaaaggacctcaggatgaccctggctcatatcaaggaccagaaagaaggcttgcattccctccaggagattagggtctgtgagatccatgaagacaacagcaccaggagctcccagcatttctactacgatggggagctctttctctcccaaaacctggagactaaggaatggacaatgccccagtcctccagagctcagaccttggccatgaacgtcaggaatttcttgaaggaagatgcaatgaagaccaagacacactatcacgctatgcatgcagactgcctgcaggaactacggcgatatctaaaatccggcgtagtcctgaggagaacagtgccccccatggtgcaggtgactcgctctgaggcctctggcggatctggggaccgtgtgacaatcacctgcagagcctcccaggacgtctccactgccgtggcgtggtaccaacagaagcccgggaaggcacccaaactgctcatttacagcgcatcctttctctactctggcgtgccgtctcgctttagcgggtccggcagcggtacagactttactctgaccatctcctctctgcaaccggaggattttgcaacctattattgccagcaatcctacacaaccccccccacctttggccagggcaccaaggtggagatcaagggaggttctagccgctccagcagctctggaggtggaggctctggcggaggaggcgaggtgcaactggtggagtctgggggcggcctggtccagcccggcggaagcttgcgcctgagctgtgccgcctccggttttaccttcaccagcactggaatctcctgggtgcgccaagctcccggcaaagggctcgaatgggtgggccgtatctaccccaccaacggaagcaccaactatgcagacagcgtgaaggggcgcttcactatctccgccgacaccagcaaaaacaccgcgtacctgcagatgaattctttgagggcagaggatactgccgtgtactactgcgcgaggacatacggcatttacgatctgtatgtggattacaccgaatacgtgatggactattggggccagggcactctggtcacagtgtctagcggtggcagctcccgcagctccagcagcggtggtggcggtagcggaggcggaggcgatatccagatgactcagagtccctcttctctgagtgcttctggcggaagtgggcagatcaccgtcacatgtcgcgcaagcggcttttatccttggaacatcaccctgagctggcggcaggacggcgtcagcctgtcccatgatacccaacagtggggagatgtgctcccggacggtcagggaacttaccagacctgggttgcaactcgcatctcccagggggaggagcagcgtttcacatgttatatggagcactctggccagcacagcactcatccggtgccgtccggaaagggatctcatcaccatcaccaccactaggatccgttgaggtctctaaaagcgtcttcctgttctcatcacatcatatcaaggttatataccatcaatattgccacagatgttacttagccttttaatatttctctaatttagtgtatatgcaatgatagttctctgatttctgagattgagtttctcatgtgtaatgattatttagagtttctctttcatctgttcaaatttttgtctagttttattttttactgatttgtaagacttctttttataatctgcatattacaattctctttactggggtgttgcaaatattttctgtcattctatggcctgacttttcttaatggttttttaattttaaaaataagtcttaatattcatgcaatctaattaacaatcttttctttgtggttaggactttgagtcataagaaatttttctctacactgaagtcatgatggcatgcttctatattattttctaaaagatttaaagttttgccttctccatttagacttataattcactggaatttttttgtgtgtatggtatgacatatgggttcccttttattttttacatataaatatatttccctgtttttctaaaaaagaaaaagatcatcattttcccattgtaaaatgccatatttttttcataggtcacttacatatatcaatgggtctgtttctgagctctactctattttatcagcctcactgtctatccccacacatctcatgctttgctctaaatcttgatatttagtggaacattctttcccattttgttctacaagaatatttttgttattgtctttgggctttctatatacattttgaaatgaggttgacaagttaataatcaacctctggattacaaaatttgtgaaagattgactggtattcttaactatgttgctccttttacgctatgtggatacgctgctttaatgcctttgtatcatgctattgcttcccgtatggctttcattttctcctccttgtataaatcctggttgctgtctctttatgaggagttgtggcccgttgtcaggcaacgtggcgtggtgtgcactgtgtttgctgacgcaacccccactggttggggcattgccaccacctgtcagctcctttccgggactttcgctttccccctccctattgccacggcggaactcatcgccgcctgccttgcccgctgctggacaggggctcggctgttgggcactgacaattccgtggtgttgtcggggaaatcatcgtcctttccttggctgctcgcctgtgttgccacctggattctgcgcgggacgtccttctgctacgtcccttcggccctcaatccagcggaccttccttcccgcggcctgctgccggctctgcggcctcttccgcctcttcgccttcgccctcagacgagtcggatctccctttgggccgcctccccgcatctgtgccttctagttgccagccatctgttgtttgcccctcccccgtgccttccttgaccctggaaggtgccactcccactgtcctttcctaataaaatgaggaaattgcatcgcattgtctgagtaggtgtcattctattctggggggtggggtggggcaggacagcaagggggaggattggcaagacaatagcaggctttgcatttttagacatttagaagcctatatcttgttacagaattggaattacacaaaaattctaccatattttgaaagcttaggttgttctgaaaaaaacaatatattgttttcctgggtaaactaaaagtcccctcgaggaaaggcccctaaagtgaaacagtgcaaaacgttcaaaaactgtctggcaatacaagttccactttgaccaaaacggctggcagtaaaagggttaagaagactgtcagccttgagcggtatcagctcactcaaaggcggtaatacggttatccacagaatcaggggataacgcaggaaagaacatgtgagcaaaaggccagcaaaaggccaggaaccgtaaaaaggccgcgttgctggcgtttttccataggctccgcccccctgacgagcatcacaaaaatcgacgctcaagtcagaggtggcgaaacccgacaggactataaagataccaggcgtttccccctggaagctccctcgtgcgctctcctgttccgaccctgccgcttaccggatacctgtccgcctttctcccttcgggaagcgtggcgctttctcatagctcacgctgtaggtatctcagttcggtgtaggtcgttcgctccaagctgggctgtgtgcacgaaccccccgttcagcccgaccgctgcgccttatccggtaactatcgtcttgagtccaacccggtaagacacgacttatcgccactggcagcagccactggtaacaggattagcagagcgaggtatgtaggcggtgctacagagttcttgaagtggtgggctaactacggctacactagaagaacagtatttggtatctgcgctctgctgaagccagttaccttcggaaaaagagttggtagctcttgatccggcaaacaaaccaccgctggtagcggtggtttttttgtttgcaagcagcagattacgcgcagaaaaaaaggatctcaagaagatcctttgatcttttctacggggtctgacgctcagtggaacgacgcgcgcgtaactcacgttaagggattttggtcatgagttagaaaaactcatcgagcatcaaatgaaactgcaatttattcatatcaggattatcaataccatatttttgaaaaagccgtttctgtaatgaaggagaaaactcaccgaggcagttccataggatggcaagatcctggtatcggtctgcgattccgactcgtccaacatcaatacaacctattaatttcccctcgtcaaaaataaggttatcaagtgagaaatcaccatgagtgacgactgaatccggtgagaatggcaaaagtttatgcatttctttccagacttgttcaacaggccagccattacgctcgtcatcaaaatcactcgcatcaaccaaaccgttattcattcgtgattgcgcctgagcgaggcgaaatacgcgatcgctgttaaaaggacaattacaaacaggaatcgagtgcaaccggcgcaggaacactgccagcgcatcaacaatattttcacctgaatcaggatattcttctaatacctggaacgctgtttttccggggatcgcagtggtgagtaaccatgcatcatcaggagtacggataaaatgcttgatggtcggaagtggcataaattccgtcagccagtttagtctgaccatctcatctgtaacatcattggcaacgctacctttgccatgtttcagaaacaactctggcgcatcgggcttcccatacaagcgatagattgtcgcacctgattgcccgacattatcgcgagcccatttatacccatataaatcagcatccatgttggaatttaatcgcggcctcgacgtttcccgttggatatggctcattttttacttcctcaccttgtcgtattatactatgccgatatactatgccgatgattaattgtcgacactgcgggggctctgtgtggtaagcaggtcttaacctttttactgccaatgacgcatgggatacgtcgtggcagtaaaagggcttaaatgccaacgacgcgtcccatacgttgttggcattttaattcttctctctgcagcggcagcatgtgccgccgctgcagagagtttctagcgatgacagcccctctgggcaacgagccgggggggctgtctttctttatgttttaaatgcactgacctcccacattccctttttagtaaaatattcagaaataatttaaatacatcattgcaatgaaaataaatgttttttattaggcagaatccagatgctcaaggcccttcataatatcccccagtttagtagttggacttagggaacaaaggaacctttaatagaaattggacagcaagaaagcgagtcaggcaccgggcttgcgggtcatgcaccaggtgcgcggtccttcgggcacctcgacgtcggcggtgacggtgaagccgagccgctcgtagaaggggaggttgcggggcgcggatgtctccaggaaggcgggcaccccggcgcgctcggccgcctccactccggggagcacgacggcgctgcccagacccttgccctggtggtcgggcgacacgccgacggtggccaggaaccacgcgggctccttgggccggtgcggcgccaggaggccttccatctgttgctgcgcggccagccgggaaccgctcaactcggccatgcgcgggccgatctcggcgaacaccgcccccgcttcgacgctctccggcgtggtccagaccgccaccgcggcgccgtcgtccgcgacccacaccttgccgatgtcgagcccgacgcgcgtgaggaagagttcttgcagctcggtgacccgctcgatgtggcggtccggatcgacggtgtggcgcgtggcggggtagtcggcgaacgcggcggcgagggtgcgtacggccctggggacgtcgtcgcgggtggcgaggcgcaccgtgggcttgtactcggtcatggtggcggacgaaaggcccggagatgaggaagaggagaacagcgcggcagacgtgcgcttttgaagcgtgcagaatgccgggcctccggaggaccttcgggcgcccgccccgcccctgagcccgcccctgagcccgcccccggacccaccccttcccagcctctgagcccagaaagcgaaggagcaaagctgctattggccgctgccccaaaggcctacccgcttccattgctcagcggtgctgtccatctgcacgagactagtgagtcgtgctacttccatttgtcacgtcctgcacgacgcgagctgcggggcgggggggaacttcctgactaggggaggagtagaaggtggcgcgaaggggccaccaaagaacggagccggttggcgcctaccggtggatgtggaatgtgtgcgaggccagaggccacttgtgtagcgccaagtgcccagcggggctgctaaagcgcatgctccagactgccttgggaaaagcgcctcccctacccggtagagaaacttgatctgtcgccgcaattcaaacttcgtgaggctccggtgcccgtcagtgacctgctatactctggagacgacttacggtaaatggcccgcctggctgaccgcccaacgacccccgcccattgacgtcaataatgacgtatgttcccatagtaacgccaatagggactttccattgacgtcaatgggtggagtatttacggtaaactgcccacttggcagtacatcaagtgtatcatatgccaagtccgccccctattgacgtcaatgacggtaaatggcccgcctggcattatgcccagtacatgaccttacgggactttcctacttggcagtacatctacgtattagtcatcgctattaccatgctgatgcggttttggcagtacaccaatgggcgtggatagcggtttgactcacggggatttccaagtctccaccccattgacgtcaatgggagtttgttttggcaccaaaatcaacgggactttccaaaatgtcgtaataaccccgccccgttgacgcaaatgggcggtaggcgtgtacggtgggaggtctatataagcagagctcgtttagtgaaccgtcagatcgcctggagaggccatccacgctgttttgacctccatagtggacaccgggaccgatccagcctccgcgtctcagg

SEQ ID NO: 66 - protein, 558 aa, Artificial Sequence
  Synthetic peptide wt MICA-Fv
EPHSLRYNLTVLSWDGSVQSGFLTEVHLDGQPFLRCDRQKCRAKPQGQWAEDVLGNKTWDRETRDLTGNGKDLRMTLAHIKDQKEGLHSLQEIRVCEIHEDNSTRSSQHFYYDGELFLSQNLETKEWTMPQSSRAQTLAMNVRNFLKEDAMKTKTHYHAMHADCLQELRRYLKSGVVLRRTVPPMVQVTRSEASGGSGDRVTITCRASQDVSTAVAWYQQKPGKAPKLLIYSASFLYSGVPSRFSGSGSGTDFTLTISSLQPEDFATYYCQQSYTTPPTFGQGTKVEIKGGSSRSSSSGGGGSGGGGEVQLVESGGGLVQPGGSLRLSCAASGFTFTSTGISWVRQAPGKGLEWVGRIYPTNGSTNYADSVKGRFTISADTSKNTAYLQMNSLRAEDTAVYYCARTYGIYDLYVDYTEYVMDYWGQGTLVTVSSGGSSRSSSSGGGGSGGGGDIQMTQSPSSLSASGGSGQITVTCRASGFYPWNITLSWRQDGVSLSHDTQQWGDVLPDGQGTYQTWVATRISQGEEQRFTCYMEHSGQHSTHPVPSGKGSHHHHHH

SEQ ID NO: 67 - protein, 558 aa, Artificial Sequence; identical to SEQ ID NO: 35
  Synthetic peptide MICwed-Fv

SEQ ID NO: 68 - protein, 558 aa, Artificial Sequence
  Synthetic peptide MICv20-Fv
EPHSLRYNLTVLSWDGSVQSGFLTEVHLDGQPFLRCDRQKCRAKPQGQWAEDVLGNKTWDRETRDLTAWGKDLRMTLAHIKDQKEGLHSLQEIRVCEIHEDNSTRSSQHFYYDGELFLSQNLETLEWTMPQSSRAQTLAMNVRNFLKEDAMQTDTHYRAMHADCLFELRRYLKSGVVLRRTVPPMVQVTRSEASGGSGDRVTITCRASQDVSTAVAWYQQKPGKAPKLLIYSASFLYSGVPSRFSGSGSGTDFTLTISSLQPEDFATYYCQQSYTTPPTFGQGTKVEIKGGSSRSSSSGGGGSGGGGEVQLVESGGGLVQPGGSLRLSCAASGFTFTSTGISWVRQAPGKGLEWVGRIYPTNGSTNYADSVKGRFTISADTSKNTAYLQMNSLRAEDTAVYYCARTYGIYDLYVDYTEYVMDYWGQGTLVTVSSGGSSRSSSSGGGGSGGGGDIQMTQSPSSLSASGGSGQITVTCRASGFYPWNITLSWRQDGVSLSHDTQQWGDVLPDGQGTYQTWVATRISQGEEQRFTCYMEHSGQHSTHPVPSGKGSHHHHHH

SEQ ID NO: 69 - protein, 558 aa, Artificial Sequence
  Synthetic peptide MICv25-Fv
EPHSLRYNLTVLSWDGSVQSGFLTEVHLDGQPFLRCDRQKCRAKPQGQWAEDVLGNKTWDRETRDLTGWGKDLRMTLAHIKDQKEGLHSLQEIRVCEIHEDNSTRSSQHFYYDGELFLSQNLETLEWTMPQSSRAQTLAMNVRNFLKEDAMETDTHYHAMRADCLSELRRYLKSGVVLRRTVPPMVQVTRSEASGGSGDRVTITCRASQDVSTAVAWYQQKPGKAPKLLIYSASFLYSGVPSRFSGSGSGTDFTLTISSLQPEDFATYYCQQSYTTPPTFGQGTKVEIKGGSSRSSSSGGGGSGGGGEVQLVESGGGLVQPGGSLRLSCAASGFTFTSTGISWVRQAPGKGLEWVGRIYPTNGSTNYADSVKGRFTISADTSKNTAYLQMNSLRAEDTAVYYCARTYGIYDLYVDYTEYVMDYWGQGTLVTVSSGGSSRSSSSGGGGSGGGGDIQMTQSPSSLSASGGSGQITVTCRASGFYPWNITLSWRQDGVSLSHDTQQWGDVLPDGQGTYQTWVATRISQGEEQRFTCYMEHSGQHSTHPVPSGKGSHHHHHH

SEQ ID NO: 70 - protein, 558 aa, Artificial Sequence
  Synthetic peptide MICv27-Fv
EPHSLRYNLTVLSWDGSVQSGFLTEVHLDGQPFLRCDRQKCRAKPQGQWAEDVLGNKTWDRETRDLTGWGKDLRMTLAHIKDQKEGLHSLQEIRVCEIHEDNSTRSSQHFYYDGELFLSQNLETLEWTMPQSSRAQTLAMNVRNFLKEDAMKTKTHYHAMRADCLSELRRYLKSGVVLRRTVPPMVQVTRSEASGGSGDRVTITCRASQDVSTAVAWYQQKPGKAPKLLIYSASFLYSGVPSRFSGSGSGTDFTLTISSLQPEDFATYYCQQSYTTPPTFGQGTKVEIKGGSSRSSSSGGGGSGGGGEVQLVESGGGLVQPGGSLRLSCAASGFTFTSTGISWVRQAPGKGLEWVGRIYPTNGSTNYADSVKGRFTISADTSKNTAYLQMNSLRAEDTAVYYCARTYGIYDLYVDYTEYVMDYWGQGTLVTVSSGGSSRSSSSGGGGSGGGGDIQMTQSPSSLSASGGSGQITVTCRASGFYPWNITLSWRQDGVSLSHDTQQWGDVLPDGQGTYQTWVATRISQGEEQRFTCYMEHSGQHSTHPVPSGKGSHHHHHH

SEQ ID NO: 71 - protein, 558 aa, Artificial Sequence
  Synthetic peptide MICv28-Fv
EPHSLRYNLTVLSWDGSVQSGFLTEVHLDGQPFLRCDRQKCRAKPQGQWAEDVLGNKTWDRETRDLTGNGKDLRMTLAHIKDQKEGLHSLQEIRVCEIHEDNSTRSSQHFYYDGELFLSQNLETLEWTMPQSSRAQTLAMNVRNFLKEDAMKTKTHYHAMRADCLSELRRYLKSGVVLRRTVPPMVQVTRSEASGGSGDRVTITCRASQDVSTAVAWYQQKPGKAPKLLIYSASFLYSGVPSRFSGSGSGTDFTLTISSLQPEDFATYYCQQSYTTPPTFGQGTKVEIKGGSSRSSSSGGGGSGGGGEVQLVESGGGLVQPGGSLRLSCAASGFTFTSTGISWVRQAPGKGLEWVGRIYPTNGSTNYADSVKGRFTISADTSKNTAYLQMNSLRAEDTAVYYCARTYGIYDLYVDYTEYVMDYWGQGTLVTVSSGGSSRSSSSGGGGSGGGGDIQMTQSPSSLSASGGSGQITVTCRASGFYPWNITLSWRQDGVSLSHDTQQWGDVLPDGQGTYQTWVATRISQGEEQRFTCYMEHSGQHSTHPVPSGKGSHHHHHH

SEQ ID NO: 72 - protein, 558 aa, Artificial Sequence; identical to SEQ ID NO: 32
  Synthetic peptide MICv42-Fv

SEQ ID NO: 73 - protein, 558 aa, Artificial Sequence
  Synthetic peptide MICv48-Fc
EPHSLRYNLTVLSWDGSVQSGFLTEVHLDGQPFLRCDRQKCRAKPQGQWAEDVLGNKTWDRETRDLTGWGKDLRMTLAHIKDQKEGLHSLQEIRVCEIHEDNSTRSSQHFYYDGELFLSQNLETLEWTMPQSSRAQTLAMNVRNFLKEDAMATDTHYIAMRADCLAELRRYLKSGVVLRRTVPPMVQVTRSEASGGSGDRVTITCRASQDVSTAVAWYQQKPGKAPKLLIYSASFLYSGVPSRFSGSGSGTDFTLTISSLQPEDFATYYCQQSYTTPPTFGQGTKVEIKGGSSRSSSSGGGGSGGGGEVQLVESGGGLVQPGGSLRLSCAASGFTFTSTGISWVRQAPGKGLEWVGRIYPTNGSTNYADSVKGRFTISADTSKNTAYLQMNSLRAEDTAVYYCARTYGIYDLYVDYTEYVMDYWGQGTLVTVSSGGSSRSSSSGGGGSGGGGDIQMTQSPSSLSASGGSGQITVTCRASGFYPWNITLSWRQDGVSLSHDTQQWGDVLPDGQGTYQTWVATRISQGEEQRFTCYMEHSGQHSTHPVPSGKGSHHHHHH

SEQ ID NO: 74 - protein, 558 aa, Artificial Sequence
  Synthetic peptide MICv49-Fv
EPHSLRYNLTVLSWDGSVQTGFLTEVHLDGQPFLRCDRQKCRAKPQGQWAEDVLGNKTWDRETRDLTQWGKDLRMTLAHIKDQKEGLHSLQEIRVCEIHEDNSTRSSQHFYYDGELFLSQNLETKEWTMPQSSRAQTLAMNVRNFLKEDAMFTDTHYRAMTADCLTELRRYLKSGVVLRRTVPPMVQVTRSEASGGSGDRVTITCRASQDVSTAVAWYQQKPGKAPKLLIYSASFLYSGVPSRFSGSGSGTDFTLTISSLQPEDFATYYCQQSYTTPPTFGQGTKVEIKGGSSRSSSSGGGGSGGGGEVQLVESGGGLVQPGGSLRLSCAASGFTFTSTGISWVRQAPGKGLEWVGRIYPTNGSTNYADSVKGRFTISADTSKNTAYLQMNSLRAEDTAVYYCARTYGIYDLYVDYTEYVMDYWGQGTLVTVSSGGSSRSSSSGGGGSGGGGDIQMTQSPSSLSASGGSGQITVTCRASGFYPWNITLSWRQDGVSLSHDTQQWGDVLPDGQGTYQTWVATRISQGEEQRFTCYMEHSGQHSTHPVPSGKGSHHHHHH

SEQ ID NO: 75 - protein, 137 aa, Artificial Sequence
  Synthetic NKG2D ectodomain
NSLFNQEVQIPLTESYCGPCPKNWICYKNNCYQFFDESKNWYESQASCMSQNASLLKVYSKEDQDLLKLVKSYHWMGLVHIPTNGSWQWEDGSILSPNLLTIIEMQKGDCALYASSFKGYIENCSTPNTYICMQRTV

SEQ ID NO: 76 - DNA, 40 bp, Artificial Sequence
  Synthetic oligonucleotide
ctgtctagagccgccaacatggggctgggcccggtcttcc

SEQ ID NO: 77 - DNA, 30 bp, Artificial Sequence
  Synthetic oligonucleotide
aacggatcctacacagtcctttgcatgcag

SEQ ID NO: 78 - DNA, 6362 bp, Artificial Sequence
  Synthetic polynucleotide, pD2509-CMV-Avi-His-natural NKG2D ectodomain
ggagagaccacacccaagctgtctagagccgccaacatggggctgggcccggtcttcctgcttctggctggcatcttcccttttgcacctccgggagctgctgctgagccccaccatcatcaccaccatggccttaacgacatcttcgaagctcaaaagatcgaatggcatgaaaactcattattcaaccaagaagttcaaattcccttgaccgaaagttactgtggcccatgtcctaaaaactggatatgttacaaaaataactgctaccaattttttgatgagagtaaaaactggtatgagagccaggcttcttgtatgtctcaaaatgccagccttctgaaagtatacagcaaagaggaccaggatttacttaaactggtgaagtcatatcattggatgggactagtacacattccaacaaatggatcttggcagtgggaagatggctccattctctcacccaacctactaacaataattgaaatgcagaagggagactgtgcactctatgcctcgagctttaaaggctatatagaaaactgttcaactccaaatacatacatctgcatgcaaaggactgtgtaggatccgttgaggtctctaaaagcgtcttcctgttctcatcacatcatatcaaggttatataccatcaatattgccacagatgttacttagccttttaatatttctctaatttagtgtatatgcaatgatagttctctgatttctgagattgagtttctcatgtgtaatgattatttagagtttctctttcatctgttcaaatttttgtctagttttattttttactgatttgtaagacttctttttataatctgcatattacaattctctttactggggtgttgcaaatattttctgtcattctatggcctgacttttcttaatggttttttaattttaaaaataagtcttaatattcatgcaatctaattaacaatcttttctttgtggttaggactttgagtcataagaaatttttctctacactgaagtcatgatggcatgcttctatattattttctaaaagatttaaagttttgccttctccatttagacttataattcactggaatttttttgtgtgtatggtatgacatatgggttcccttttattttttacatataaatatatttccctgtttttctaaaaaagaaaaagatcatcattttcccattgtaaaatgccatatttttttcataggtcacttacatatatcaatgggtctgtttctgagctctactctattttatcagcctcactgtctatccccacacatctcatgctttgctctaaatcttgatatttagtggaacattctttcccattttgttctacaagaatatttttgttattgtctttgggctttctatatacattttgaaatgaggttgacaagttaataatcaacctctggattacaaaatttgtgaaagattgactggtattcttaactatgttgctccttttacgctatgtggatacgctgctttaatgcctttgtatcatgctattgcttcccgtatggctttcattttctcctccttgtataaatcctggttgctgtctctttatgaggagttgtggcccgttgtcaggcaacgtggcgtggtgtgcactgtgtttgctgacgcaacccccactggttggggcattgccaccacctgtcagctcctttccgggactttcgctttccccctccctattgccacggcggaactcatcgccgcctgccttgcccgctgctggacaggggctcggctgttgggcactgacaattccgtggtgttgtcggggaaatcatcgtcctttccttggctgctcgcctgtgttgccacctggattctgcgcgggacgtccttctgctacgtcccttcggccctcaatccagcggaccttccttcccgcggcctgctgccggctctgcggcctcttccgcctcttcgccttcgccctcagacgagtcggatctccctttgggccgcctccccgcatctgtgccttctagttgccagccatctgttgtttgcccctcccccgtgccttccttgaccctggaaggtgccactcccactgtcctttcctaataaaatgaggaaattgcatcgcattgtctgagtaggtgtcattctattctggggggtggggtggggcaggacagcaagggggaggattggcaagacaatagcaggctttgcatttttagacatttagaagcctatatcttgttacagaattggaattacacaaaaattctaccatattttgaaagcttaggttgttctgaaaaaaacaatatattgttttcctgggtaaactaaaagtcccctcgaggaaaggcccctaaagtgaaacagtgcaaaacgttcaaaaactgtctggcaatacaagttccactttgaccaaaacggctggcagtaaaagggttaagaagactgtcagccttgagcggtatcagctcactcaaaggcggtaatacggttatccacagaatcaggggataacgcaggaaagaacatgtgagcaaaaggccagcaaaaggccaggaaccgtaaaaaggccgcgttgctggcgtttttccataggctccgcccccctgacgagcatcacaaaaatcgacgctcaagtcagaggtggcgaaacccgacaggactataaagataccaggcgtttccccctggaagctccctcgtgcgctctcctgttccgaccctgccgcttaccggatacctgtccgcctttctcccttcgggaagcgtggcgctttctcatagctcacgctgtaggtatctcagttcggtgtaggtcgttcgctccaagctgggctgtgtgcacgaaccccccgttcagcccgaccgctgcgccttatccggtaactatcgtcttgagtccaacccggtaagacacgacttatcgccactggcagcagccactggtaacaggattagcagagcgaggtatgtaggcggtgctacagagttcttgaagtggtgggctaactacggctacactagaagaacagtatttggtatctgcgctctgctgaagccagttaccttcggaaaaagagttggtagctcttgatccggcaaacaaaccaccgctggtagcggtggtttttttgtttgcaagcagcagattacgcgcagaaaaaaaggatctcaagaagatcctttgatcttttctacggggtctgacgctcagtggaacgacgcgcgcgtaactcacgttaagggattttggtcatgagttagaaaaactcatcgagcatcaaatgaaactgcaatttattcatatcaggattatcaataccatatttttgaaaaagccgtttctgtaatgaaggagaaaactcaccgaggcagttccataggatggcaagatcctggtatcggtctgcgattccgactcgtccaacatcaatacaacctattaatttcccctcgtcaaaaataaggttatcaagtgagaaatcaccatgagtgacgactgaatccggtgagaatggcaaaagtttatgcatttctttccagacttgttcaacaggccagccattacgctcgtcatcaaaatcactcgcatcaaccaaaccgttattcattcgtgattgcgcctgagcgaggcgaaatacgcgatcgctgttaaaaggacaattacaaacaggaatcgagtgcaaccggcgcaggaacactgccagcgcatcaacaatattttcacctgaatcaggatattcttctaatacctggaacgctgtttttccggggatcgcagtggtgagtaaccatgcatcatcaggagtacggataaaatgcttgatggtcggaagtggcataaattccgtcagccagtttagtctgaccatctcatctgtaacatcattggcaacgctacctttgccatgtttcagaaacaactctggcgcatcgggcttcccatacaagcgatagattgtcgcacctgattgcccgacattatcgcgagcccatttatacccatataaatcagcatccatgttggaatttaatcgcggcctcgacgtttcccgttggatatggctcattttttacttcctcaccttgtcgtattatactatgccgatatactatgccgatgattaattgtcgacactgcgggggctctgtgtggtaagcaggtcttaacctttttactgccaatgacgcatgggatacgtcgtggcagtaaaagggcttaaatgccaacgacgcgtcccatacgttgttggcattttaattcttctctctgcagcggcagcatgtgccgccgctgcagagagtttctagcgatgacagcccctctgggcaacgagccgggggggctgtctttctttatgttttaaatgcactgacctcccacattccctttttagtaaaatattcagaaataatttaaatacatcattgcaatgaaaataaatgttttttattaggcagaatccagatgctcaaggcccttcataatatcccccagtttagtagttggacttagggaacaaaggaacctttaatagaaattggacagcaagaaagcgagtcaggcaccgggcttgcgggtcatgcaccaggtgcgcggtccttcgggcacctcgacgtcggcggtgacggtgaagccgagccgctcgtagaaggggaggttgcggggcgcggatgtctccaggaaggcgggcaccccggcgcgctcggccgcctccactccggggagcacgacggcgctgcccagacccttgccctggtggtcgggcgacacgccgacggtggccaggaaccacgcgggctccttgggccggtgcggcgccaggaggccttccatctgttgctgcgcggccagccgggaaccgctcaactcggccatgcgcgggccgatctcggcgaacaccgcccccgcttcgacgctctccggcgtggtccagaccgccaccgcggcgccgtcgtccgcgacccacaccttgccgatgtcgagcccgacgcgcgtgaggaagagttcttgcagctcggtgacccgctcgatgtggcggtccggatcgacggtgtggcgcgtggcggggtagtcggcgaacgcggcggcgagggtgcgtacggccctggggacgtcgtcgcgggtggcgaggcgcaccgtgggcttgtactcggtcatggtggcggacgaaaggcccggagatgaggaagaggagaacagcgcggcagacgtgcgcttttgaagcgtgcagaatgccgggcctccggaggaccttcgggcgcccgccccgcccctgagcccgcccctgagcccgcccccggacccaccccttcccagcctctgagcccagaaagcgaaggagcaaagctgctattggccgctgccccaaaggcctacccgcttccattgctcagcggtgctgtccatctgcacgagactagtgagtcgtgctacttccatttgtcacgtcctgcacgacgcgagctgcggggcgggggggaacttcctgactaggggaggagtagaaggtggcgcgaaggggccaccaaagaacggagccggttggcgcctaccggtggatgtggaatgtgtgcgaggccagaggccacttgtgtagcgccaagtgcccagcggggctgctaaagcgcatgctccagactgccttgggaaaagcgcctcccctacccggtagagaaacttgatctgtcgccgcaattcaaacttcgtgaggctccggtgcccgtcagtgacctgctatactctggagacgacttacggtaaatggcccgcctggctgaccgcccaacgacccccgcccattgacgtcaataatgacgtatgttcccatagtaacgccaatagggactttccattgacgtcaatgggtggagtatttacggtaaactgcccacttggcagtacatcaagtgtatcatatgccaagtccgccccctattgacgtcaatgacggtaaatggcccgcctggcattatgcccagtacatgaccttacgggactttcctacttggcagtacatctacgtattagtcatcgctattaccatgctgatgcggttttggcagtacaccaatgggcgtggatagcggtttgactcacggggatttccaagtctccaccccattgacgtcaatgggagtttgttttggcaccaaaatcaacgggactttccaaaatgtcgtaataaccccgccccgttgacgcaaatgggcggtaggcgtgtacggtgggaggtctatataagcagagctcgtttagtgaaccgtcagatcgcctggagaggccatccacgctgttttgacctccatagtggacaccgggaccgatccagcctccgcgtctcagg

SEQ ID NO: 79 - protein, 160 aa, Artificial Sequence
  Synthetic peptide, His-avitag-natural NKG2D ectodomain
EPHHHHHHGLNDIFEAQKIEWHENSLFNQEVQIPLTESYCGPCPKNWICYKNNCYQFFDESKNWYESQASCMSQNASLLKVYSKEDQDLLKLVKSYHWMGLVHIPTNGSWQWEDGSILSPNLLTIIEMQKGDCALYASSFKGYIENCSTPNTYICMQRTV

SEQ ID NO: 80 - protein, 160 aa, Artificial Sequence
  Synthetic peptide, His-avitag-non-natural NKG2D Y152A ectodomain
EPHHHHHHGLNDIFEAQKIEWHENSLFNQEVQIPLTESYCGPCPKNWICYKNNCYQFFDESKNWYESQASCMSQNASLLKVYSKEDQDLLKLVKSAHWMGLVHIPTNGSWQWEDGSILSPNLLTIIEMQKGDCALYASSFKGYIENCSTPNTYICMQRTV

SEQ ID NO: 81 - protein, 160 aa, Artificial Sequence
  Synthetic peptide, His-avitag-non-natural NKG2D Y199A ectodomain
EPHHHHHHGLNDIFEAQKIEWHENSLFNQEVQIPLTESYCGPCPKNWICYKNNCYQFFDESKNWYESQASCMSQNASLLKVYSKEDQDLLKLVKSYHWMGLVHIPTNGSWQWEDGSILSPNLLTIIEMQKGDCALYASSFKGAIENCSTPNTYICMQRTV

SEQ ID NO: 82 - protein, 160 aa, Artificial Sequence
  Synthetic peptide, His-avitag-non-natural NKG2D Y152A +Y199A ectodomain
EPHHHHHHGLNDIFEAQKIEWHENSLFNQEVQIPLTESYCGPCPKNWICYKNNCYQFFDESKNWYESQASCMSQNASLLKVYSKEDQDLLKLVKSAHWMGLVHIPTNGSWQWEDGSILSPNLLTIIEMQKGDCALYASSFKGAIENCSTPNTYICMQRTV

SEQ ID NO: 83 - DNA, 7640 bp, Artificial Sequence
  Synthetic polynucleotide, wt MIC-Fc expression vector
ggagagaccacacccaagctgtctagagccgccaacatggggctgggcccggtcttcctgcttctggctggcatcttcccttttgcacctccgggagctgctgctgagccccacagtcttcgttataacctcacggtgctgtcctgggatggatctgtgcagtcagggtttctcactgaggtacatctggatggtcagcccttcctgcgctgtgacaggcagaaatgcagggcaaagccccagggacagtgggcagaagatgtcctgggaaataagacatgggacagagagaccagagacttgacagggtggggaaaggacctcaggatgaccctggctcatatcaaggaccagaaagaaggcttgcattccctccaggagattagggtctgtgagatccatgaagacaacagcaccaggagctcccagcatttctactacgatggggagctctttctctcccaaaacctggagactaaggaatggacaatgccccagtcctccagagctcagaccttggccatgaacgtcaggaatttcttgaaggaagatgcaatggagaccgatacacactatcacgctatgcatgcagactgcctgcaggaactacggcgatatctaaaatccggcgtagtcctgaggagaacagtgccccccatggtgaatgtcacccgcagcgaggcctcagagggcaacattaccgtgacatgcagggcttctggcttctatccctggaatatcacactgagctggcgtcaggatggggtatctttgagccacgacacccagcagtggggggatgtcctgcctgatgggaatggaacctaccagacctgggtggccaccaggatttgccaaggagaggagcagaggttcacctgctacatggaacacagcgggaatcacagcactcaccctgtgccctctgggaaaatcgaaggacgcatggacccaaagagttgcgacaaaactcacacatgcccaccgtgcccaggtaagccagcccaggcctcgccctccagctcaaggcgggacaggtgccctagagtagcctgcatccagggacaggccccagccgggtgctgacacgtccacctccatctcttcctcagcacctgaactcctggggggaccgtcagtcttcctcttccccccaaaacccaaggacaccctcatgatctcccggacccctgaggtcacatgcgtggtggtggacgtgagccacgaagaccctgaggtcaagttcaactggtacgtggacggcgtggaggtgcataatgccaagacaaagccgcgggaggagcagtacaacagcacgtaccgtgtggtcagcgtcctcaccgtcctgcaccaggactggctgaatggcaaggagtacaagtgcaaggtctccaacaaagccctcccagcccccatcgagaaaaccatctccaaagccaaaggtgggacccgtggggtgcgagggccacatggacagaggccggctcggcccaccctctgccctgagagtgactgctgtaccaacctctgtccctacagggcagccccgagaaccacaggtgtacaccctgcccccatcccgggatgagctgaccaagaaccaggtcagcctgacctgcctggtcaaaggcttctatcccagcgacatcgccgtggagtgggagagcaatgggcagccggagaacaactacaagaccacgcctcccgtgctggactccgacggctccttcttcctctacagcaagctcaccgtggacaagagcaggtggcagcaggggaacgtcttctcatgctccgtgatgcatgaggctctgcacaaccactacacgcagaagagcctctccctgtctccgggtaaatgataggatccggttgaggtctctaaaagcgtcttcctgttctcatcacatcatatcaaggttatataccatcaatattgccacagatgttacttagccttttaatatttctctaatttagtgtatatgcaatgatagttctctgatttctgagattgagtttctcatgtgtaatgattatttagagtttctctttcatctgttcaaatttttgtctagttttattttttactgatttgtaagacttctttttataatctgcatattacaattctctttactggggtgttgcaaatattttctgtcattctatggcctgacttttcttaatggttttttaattttaaaaataagtcttaatattcatgcaatctaattaacaatcttttctttgtggttaggactttgagtcataagaaatttttctctacactgaagtcatgatggcatgcttctatattattttctaaaagatttaaagttttgccttctccatttagacttataattcactggaatttttttgtgtgtatggtatgacatatgggttcccttttattttttacatataaatatatttccctgtttttctaaaaaagaaaaagatcatcattttcccattgtaaaatgccatatttttttcataggtcacttacatatatcaatgggtctgtttctgagctctactctattttatcagcctcactgtctatccccacacatctcatgctttgctctaaatcttgatatttagtggaacattctttcccattttgttctacaagaatatttttgttattgtctttgggctttctatatacattttgaaatgaggttgacaagttaataatcaacctctggattacaaaatttgtgaaagattgactggtattcttaactatgttgctccttttacgctatgtggatacgctgctttaatgcctttgtatcatgctattgcttcccgtatggctttcattttctcctccttgtataaatcctggttgctgtctctttatgaggagttgtggcccgttgtcaggcaacgtggcgtggtgtgcactgtgtttgctgacgcaacccccactggttggggcattgccaccacctgtcagctcctttccgggactttcgctttccccctccctattgccacggcggaactcatcgccgcctgccttgcccgctgctggacaggggctcggctgttgggcactgacaattccgtggtgttgtcggggaaatcatcgtcctttccttggctgctcgcctgtgttgccacctggattctgcgcgggacgtccttctgctacgtcccttcggccctcaatccagcggaccttccttcccgcggcctgctgccggctctgcggcctcttccgcctcttcgccttcgccctcagacgagtcggatctccctttgggccgcctccccgcatctgtgccttctagttgccagccatctgttgtttgcccctcccccgtgccttccttgaccctggaaggtgccactcccactgtcctttcctaataaaatgaggaaattgcatcgcattgtctgagtaggtgtcattctattctggggggtggggtggggcaggacagcaagggggaggattggcaagacaatagcaggctttgcatttttagacatttagaagcctatatcttgttacagaattggaattacacaaaaattctaccatattttgaaagcttaggttgttctgaaaaaaacaatatattgttttcctgggtaaactaaaagtcccctcgaggaaaggcccctaaagtgaaacagtgcaaaacgttcaaaaactgtctggcaatacaagttccactttgaccaaaacggctggcagtaaaagggttaagaagactgtcagccttgagcggtatcagctcactcaaaggcggtaatacggttatccacagaatcaggggataacgcaggaaagaacatgtgagcaaaaggccagcaaaaggccaggaaccgtaaaaaggccgcgttgctggcgtttttccataggctccgcccccctgacgagcatcacaaaaatcgacgctcaagtcagaggtggcgaaacccgacaggactataaagataccaggcgtttccccctggaagctccctcgtgcgctctcctgttccgaccctgccgcttaccggatacctgtccgcctttctcccttcgggaagcgtggcgctttctcatagctcacgctgtaggtatctcagttcggtgtaggtcgttcgctccaagctgggctgtgtgcacgaaccccccgttcagcccgaccgctgcgccttatccggtaactatcgtcttgagtccaacccggtaagacacgacttatcgccactggcagcagccactggtaacaggattagcagagcgaggtatgtaggcggtgctacagagttcttgaagtggtgggctaactacggctacactagaagaacagtatttggtatctgcgctctgctgaagccagttaccttcggaaaaagagttggtagctcttgatccggcaaacaaaccaccgctggtagcggtggtttttttgtttgcaagcagcagattacgcgcagaaaaaaaggatctcaagaagatcctttgatcttttctacggggtctgacgctcagtggaacgacgcgcgcgtaactcacgttaagggattttggtcatgagttagaaaaactcatcgagcatcaaatgaaactgcaatttattcatatcaggattatcaataccatatttttgaaaaagccgtttctgtaatgaaggagaaaactcaccgaggcagttccataggatggcaagatcctggtatcggtctgcgattccgactcgtccaacatcaatacaacctattaatttcccctcgtcaaaaataaggttatcaagtgagaaatcaccatgagtgacgactgaatccggtgagaatggcaaaagtttatgcatttctttccagacttgttcaacaggccagccattacgctcgtcatcaaaatcactcgcatcaaccaaaccgttattcattcgtgattgcgcctgagcgaggcgaaatacgcgatcgctgttaaaaggacaattacaaacaggaatcgagtgcaaccggcgcaggaacactgccagcgcatcaacaatattttcacctgaatcaggatattcttctaatacctggaacgctgtttttccggggatcgcagtggtgagtaaccatgcatcatcaggagtacggataaaatgcttgatggtcggaagtggcataaattccgtcagccagtttagtctgaccatctcatctgtaacatcattggcaacgctacctttgccatgtttcagaaacaactctggcgcatcgggcttcccatacaagcgatagattgtcgcacctgattgcccgacattatcgcgagcccatttatacccatataaatcagcatccatgttggaatttaatcgcggcctcgacgtttcccgttggatatggctcattttttacttcctcaccttgtcgtattatactatgccgatatactatgccgatgattaattgtcgacactgcgggggctctgtgtggtaagcaggtcttaacctttttactgccaatgacgcatgggatacgtcgtggcagtaaaagggcttaaatgccaacgacgcgtcccatacgttgttggcattttaattcttctctctgcagcggcagcatgtgccgccgctgcagagagtttctagcgatgacagcccctctgggcaacgagccgggggggctgtctttctttatgttttaaatgcactgacctcccacattccctttttagtaaaatattcagaaataatttaaatacatcattgcaatgaaaataaatgttttttattaggcagaatccagatgctcaaggcccttcataatatcccccagtttagtagttggacttagggaacaaaggaacctttaatagaaattggacagcaagaaagcgagtcaggcaccgggcttgcgggtcatgcaccaggtgcgcggtccttcgggcacctcgacgtcggcggtgacggtgaagccgagccgctcgtagaaggggaggttgcggggcgcggatgtctccaggaaggcgggcaccccggcgcgctcggccgcctccactccggggagcacgacggcgctgcccagacccttgccctggtggtcgggcgacacgccgacggtggccaggaaccacgcgggctccttgggccggtgcggcgccaggaggccttccatctgttgctgcgcggccagccgggaaccgctcaactcggccatgcgcgggccgatctcggcgaacaccgcccccgcttcgacgctctccggcgtggtccagaccgccaccgcggcgccgtcgtccgcgacccacaccttgccgatgtcgagcccgacgcgcgtgaggaagagttcttgcagctcggtgacccgctcgatgtggcggtccggatcgacggtgtggcgcgtggcggggtagtcggcgaacgcggcggcgagggtgcgtacggccctggggacgtcgtcgcgggtggcgaggcgcaccgtgggcttgtactcggtcatggtggcggacgaaaggcccggagatgaggaagaggagaacagcgcggcagacgtgcgcttttgaagcgtgcagaatgccgggcctccggaggaccttcgggcgcccgccccgcccctgagcccgcccctgagcccgcccccggacccaccccttcccagcctctgagcccagaaagcgaaggagcaaagctgctattggccgctgccccaaaggcctacccgcttccattgctcagcggtgctgtccatctgcacgagactagtgagtcgtgctacttccatttgtcacgtcctgcacgacgcgagctgcggggcgggggggaacttcctgactaggggaggagtagaaggtggcgcgaaggggccaccaaagaacggagccggttggcgcctaccggtggatgtggaatgtgtgcgaggccagaggccacttgtgtagcgccaagtgcccagcggggctgctaaagcgcatgctccagactgccttgggaaaagcgcctcccctacccggtagagaaacttgatctgtcgccgcaattcaaacttcgtgaggctccggtgcccgtcagtgacctgctatactctggagacgacttacggtaaatggcccgcctggctgaccgcccaacgacccccgcccattgacgtcaataatgacgtatgttcccatagtaacgccaatagggactttccattgacgtcaatgggtggagtatttacggtaaactgcccacttggcagtacatcaagtgtatcatatgccaagtccgccccctattgacgtcaatgacggtaaatggcccgcctggcattatgcccagtacatgaccttacgggactttcctacttggcagtacatctacgtattagtcatcgctattaccatgctgatgcggttttggcagtacaccaatgggcgtggatagcggtttgactcacggggatttccaagtctccaccccattgacgtcaatgggagtttgttttggcaccaaaatcaacgggactttccaaaatgtcgtaataaccccgccccgttgacgcaaatgggcggtaggcgtgtacggtgggaggtctatataagcagagctcgtttagtgaaccgtcagatcgcctggagaggccatccacgctgttttgacctccatagtggacaccgggaccgatccagcctccgcgtctcagg

SEQ ID NO: 84 - protein, 438 aa, Artificial Sequence
  Synthetic peptide, MICA-Fc
EPHSLRYNLTVLSWDGSVQSGFLTEVHLDGQPFLRCDRQKCRAKPQGQWAEDVLGNKTWDRETRDLTGNGKDLRMTLAHIKDQKEGLHSLQEIRVCEIHEDNSTRSSQHFYYDGELFLSQNLETKEWTMPQSSRAQTLAMNVRNFLKEDAMKTKTHYHAMHADCLQELRRYLKSGVVLRRTVPPMVNVTRSEASEGNITVTCRASGFYPWNITLSWRQDGVSLSHDTQQWGDVLPDGNGTYQTWVATRISQGEEQRFTCYMEHSGNHSTHPVPSGKIEGRMDPKSCDKTHTCPPCPAPELLGGPSVFLFPPKPKDTLMISRTPEVTCVVVDVSHEDPEVKFNWYVDGVEVHNAKTKPREEQYNSTYRVVSVLTVLHQDWLNGKEYKCKVSNKALPAPIEKTISKAKGQPREPQVYTLPPSRDELTKNQVSLTCLVKGF

SEQ ID NO: 85 - protein, 513 aa, Artificial Sequence
  Synthetic peptide, MICwed-Fc
EPHSLRYNLTVLSWDGSVQSGFLTEVHLDGQPFLRCDRQKCRAKPQGQWAEDVLGNKTWDRETRDLTGWGKDLRMTLAHIKDQKEGLHSLQEIRVCEIHEDNSTRSSQHFYYDGELFLSQNLETKEWTMPQSSRAQTLAMNVRNFLKEDAMETDTHYHAMHADCLQELRRYLKSGVVLRRTVPPMVNVTRSEASEGNITVTCRASGFYPWNITLSWRQDGVSLSHDTQQWGDVLPDGNGTYQTWVATRISQGEEQRFTCYMEHSGNHSTHPVPSGKIEGRMDPKSCDKTHTCPPCPAPELLGGPSVFLFPPKPKDTLMISRTPEVTCVVVDVSHEDPEVKFNWYVDGVEVHNAKTKPREEQYNSTYRVVSVLTVLHQDWLNGKEYKCKVSNKALPAPIEKTISKAKGQPREPQVYTLPPSRDELTKNQVSLTCLVKGFYPSDIAVEWESNGQPENNYKTTPPVLDSDGSFFLYSKLTVDKSRWQQGNVFSCSVMHEALHNHYTQKSLSLSPGK

SEQ ID NO: 86 - protein, 513 aa, Artificial Sequence
  Synthetic peptide, MICv25-Fc
EPHSLRYNLTVLSWDGSVQSGFLTEVHLDGQPFLRCDRQKCRAKPQGQWAEDVLGNKTWDRETRDLTGWGKDLRMTLAHIKDQKEGLHSLQEIRVCEIHEDNSTRSSQHFYYDGELFLSQNLETLEWTMPQSSRAQTLAMNVRNFLKEDAMETDTHYHAMRADCLSELRRYLKSGVVLRRTVPPMVNVTRSEASEGNITVTCRASGFYPWNITLSWRQDGVSLSHDTQQWGDVLPDGNGTYQTWVATRISQGEEQRFTCYMEHSGNHSTHPVPSGKIEGRMDPKSCDKTHTCPPCPAPELLGGPSVFLFPPKPKDTLMISRTPEVTCVVVDVSHEDPEVKFNWYVDGVEVHNAKTKPREEQYNSTYRVVSVLTVLHQDWLNGKEYKCKVSNKALPAPIEKTISKAKGQPREPQVYTLPPSRDELTKNQVSLTCLVKGFYPSDIAVEWESNGQPENNYKTTPPVLDSDGSFFLYSKLTVDKSRWQQGNVFSCSVMHEALHNHYTQKSLSLSPGK

SEQ ID NO: 87 - protein, 186 aa, Artificial Sequence
  Synthetic peptide, ULBP2 R80W
AAEPHSLSYDITVIPKFRPGPRWCAVQGQVDEKTFLHYDCGNKTVTPVSPLGKKLNVTTAWKAQNPVLREVVDILTEQLWDIQLENYTPKEPLTLQARMSCEQKAEGHSSGSWQFSFDGQIFLLFDSEKRMWTTVHPGARKMKEKWENDKVVAMSFHYFSMGDCIGWLEDFLMGMDSTLEPSAGAP

SEQ ID NO: 88 - protein, 186 aa, Artificial Sequence
  Synthetic peptide, ULBP2 V151D
AAEPHSLSYDITVIPKFRPGPRWCAVQGQVDEKTFLHYDCGNKTVTPVSPLGKKLNVTTAWKAQNPVLREVVDILTEQLRDIQLENYTPKEPLTLQARMSCEQKAEGHSSGSWQFSFDGQIFLLFDSEKRMWTTVHPGARKMKEKWENDKDVAMSFHYFSMGDCIGWLEDFLMGMDSTLEPSAGAP

SEQ ID NO: 89 - protein, 184 aa, Artificial Sequence
  Synthetic peptide, ULBP3 R162G
AAEPHSLWYNFTIIHLPRHGQQWCEVQSQVDQKNFLSYDCGSDKVLSMGHLEEQLYATDAWGKQLEMLREVGQRLRLELADTELEDFTPSGPLTLQVRMSCESEADGYIRGSWQFSFDGRKFLLFDSNNRKWTVVHAGARRMKEKWEKDSGLTTFFKMVSMGDCKSWLRDFLMHRKKRLEPTAP

SEQ ID NO: 90 - protein, 182 aa, Artificial Sequence
  Synthetic peptide, MICA25.17
EPHSLRYNLTVLSWDGSVQSGFLTEVHLDGQPFLRCDRQKCRAKPQGQWAEDVLGNKTWDRETRDLTGWGTTLLMTLAHIKDQKEGLHSLQEIRVCEIHEDNSTRSSQHFYYDGELFLSQNLETLEWTMPQSSRAQTLAMNVRNFLKEDAMETDIGYRLMRADCLSELRRYLKSGVVLRRTV

SEQ ID NO: 91 - protein, 182 aa, Artificial Sequence
  Synthetic peptide, MICA25.18
EPHSLRYNLTVLSWDGSVQSGFLTEVHLDGQPFLRCDRQKCRAKPQGQWAEDVLGNKTWDRETRDLTGWGTFLRMTLAHIKDQKEGLHSLQEIRVCEIHEDNSTRSSQHFYYDGELFLSQNLETLEWTMPQSSRAQTLAMNVRNFLKEDAMETDRSGLLMRADCLSELRRYLKSGVVLRRTV

SEQ ID NO: 92 - protein, 186 aa, Artificial Sequence
  Synthetic peptide, ULBP2.S1
AAEPHSLSYDITVIPKFRPGPRWCAVQGQVDEKTFLHYDCGNKTVTPVSPLGKKLNVTTAWKAQNPVLREVVDILTEQLWDIQLENYTPKEPLTLQARMSCEQKAEGHSSGSWQFSFDGQIFLLFDSEKRMWTTVHPGARKMKEKWENDKVVATTLYTWSMGDCIGWLEDFLMGMDSTLEPSAGAP

SEQ ID NO: 93 - protein, 186 aa, Artificial Sequence
  Synthetic peptide, ULBP2.S2
AAEPHSLSYDITVIPKFRPGPRWCAVQGQVDEKTFLHYDCGNKTVTPVSPLGKKLNVTTAWKAQNPVLREVVDILTEQLWDIQLENYTPKEPLTLQARMSCEQKAEGHSSGSWQFSFDGQIFLLFDSEKRMWTTVHPGARKMKEKWENDKVVATLMRIWSMGDCIGWLEDFLMGMDSTLEPSAGAP

SEQ ID NO: 94 - protein, 186 aa, Artificial Sequence
  Synthetic peptide, ULBP2.S3
AAEPHSLSYDITVIPKFRPGPRWCAVQGQVDEKTFLHYDCGNKTVTPVSPLGKKLNVTTAWKAQNPVLREVVDILTEQLWDIQLENYTPKEPLTLQARMSCEQKAEGHSSGSWQFSFDGQIFLLFDSEKRMWTTVHPGARKMKEKWENDKVVATKLYLWSMGDCIGWLEDFLMGMDSTLEPSAGAP

SEQ ID NO: 95 - protein, 184 aa, Artificial Sequence
  Synthetic peptide, ULBP3.S1
AAEPHSLWYNFTIIHLPRHGQQWCEVQSQVDQKNFLSYDCGSDKVLSMGHLEEQLYATDAWGKQLEMLREVGQRLRLELADTELEDFTPSGPLTLQVRMSCESEADGYIRGSWQFSFDGRKFLLFDSNNRKWTVVHAGARRMKEKWEKDSGLTTDLIRRSMGDCKSWLRDFLMHRKKRLEPTAP

SEQ ID NO: 96 - protein, 184 aa, Artificial Sequence
  Synthetic peptide ULBP3.S2
AAEPHSLWYNFTIIHLPRHGQQWCEVQSQVDQKNFLSYDCGSDKVLSMGHLEEQLYATDAWGKQLEMLREVGQRLRLELADTELEDFTPSGPLTLQVRMSCESEADGYIRGSWQFSFDGRKFLLFDSNNRKWTVVHAGARRMKEKWEKDSGLTTYFYLRSMGDCKSWLRDFLMHRKKRLEPTAP

SEQ ID NO: 97 - protein, 657 aa, Artificial Sequence
  Synthetic peptide, R3 HC25.17
MRPIVLVLLFATSALAEVQLVESGGGLVQPGGSLRLSCAASGFTFTSTGISWVRQAPGKGLEWVGRIYPTNGSTNYADSVKGRFTISADTSKNTAYLQMNSLRAEDTAVYYCARTYGIYDLYVDYTEYVMDYWGQGTLVTVSSASTKGPSVFPLAPSSKSTSGGTAALGCLVKDYFPEPVTVSWNSGALTSGVHTFPAVLQSSGLYSLSSVVTVPSSSLGTQTYICNVNHKPSNTKVDKKVEPKSCDKTHTCPPCPAPELLGGPSVFLFPPKPKDTLMISRTPEVTCVVVDVSHEDPEVKFNWYVDGVEVHNAKTKPREEQYNSTYRVVSVLTVLHQDWLNGKEYKCKVSNKALPAPIEKTISKAKGQPREPQVYTLPPSRDELTKNQVSLTCLVKGFYPSDIAVEWESNGQPENNYKTTPPVLDSDGSFFLYSKLTVDKSRWQQGNVFSCSVMHEALHNHYTQKSLSLSPGGGGSEPHSLRYNLTVLSWDGSVQSGFLTEVHLDGQPFLRCDRQKCRAKPQGQWAEDVLGNKTWDRETRDLTGWGTTLLMTLAHIKDQKEGLHSLQEIRVCEIHEDNSTRSSQHFYYDGELFLSQNLETLEWTMPQSSRAQTLAMNVRNFLKEDAMETDIGYRLMRADCLSELRRYLKSGVVLRRT

SEQ ID NO: 98 - protein, 656 aa, Artificial Sequence
  Synthetic peptide, R3 HC.U2S3
MRPIVLVLLFATSALAEVQLVESGGGLVQPGGSLRLSCAASGFTFTSTGISWVRQAPGKGLEWVGRIYPTNGSTNYADSVKGRFTISADTSKNTAYLQMNSLRAEDTAVYYCARTYGIYDLYVDYTEYVMDYWGQGTLVTVSSASTKGPSVFPLAPSSKSTSGGTAALGCLVKDYFPEPVTVSWNSGALTSGVHTFPAVLQSSGLYSLSSVVTVPSSSLGTQTYICNVNHKPSNTKVDKKVEPKSCDKTHTCPPCPAPELLGGPSVFLFPPKPKDTLMISRTPEVTCVVVDVSHEDPEVKFNWYVDGVEVHNAKTKPREEQYNSTYRVVSVLTVLHQDWLNGKEYKCKVSNKALPAPIEKTISKAKGQPREPQVYTLPPSRDELTKNQVSLTCLVKGFYPSDIAVEWESNGQPENNYKTTPPVLDSDGSFFLYSKLTVDKSRWQQGNVFSCSVMHEALHNHYTQKSLSLSPGGGGSEPHSLSYDITVIPKFRPGPRWCAVQGQVDEKTFLHYDCGNKTVTPVSPLGKKLNVTTAWKAQNPVLREVVDILTEQLWDIQLENYTPKEPLTLQARMSCEQKAEGHSSGSWQFSFDGQIFLLFDSEKRMWTTVHPGARKMKEKWENDKVVATKLYLWSMGDCIGWLEDFLMGMDSTLEPS

SEQ ID NO: 99 - protein, 171 aa, Homo sapiens MICA
HSLRYNLTVLSGDGSVQSGFLAEVHLDGQPFLRCDRQKCRAKPQGQWAEDVLGNKTWDRETRDLTGNGKDLRMTLAHIKDQKEGLHSLQEIRVCEIHEDNSTRSSQHFYYDGELFLSQNLETEEWTMPQSSRAQTLAMNVRNFLKEDAMKTKTHYHAMHADCLQELRRYLK

SEQ ID NO: 100 - protein, 169 aa, Homo sapiens ULBP1
HCLCYDFIITPKSRPEPQWCEVQGLVDERPFLHYDCVNHKAKAFASLGKKVNVTKTWEEQTETLRDVVDFLKGQLLDIQVENLIPIEPLTLQARMSCEHEAHGHGRGSWQFLFNGQKFLLFDSNNRKWTALHPGAKKMTEKWEKNRDVTMFFQKISLGDCKMWLEEFLM

SEQ ID NO: 101 - protein, 169 aa, Homo sapiens ULBP2
HSLCYDITVIPKFRPGPRWCAVQGQVDEKTFLHYDCGNKTVTPVSPLGKKLNVTTAWKAQNPVLREVVDILTEQLRDIQLENYTPKEPLTLQARMSCEQKAEGHSSGSWQFSFDGQIFLLFDSEKRMWTTVHPGARKMKEKWENDKVVAMSFHYFSMGDCIGWLEDFLM

SEQ ID NO: 102 - protein, 169 aa, Homo sapiens ULBP3
HSLWYNFTIIHLPRHGQQWCEVQSQVDQKNFLSYDCGSDKVLSMGHLEEQLYATDAWGKQLEMLREVGQRLRLELADTELEDFTPSGPLTLQVRMSCECEADGYIRGSWQFSFDGRKFLLFDSNNRKWTVVHAGARRMKEKWEKDSGLTTFFKMVSMRDCKSWLRDFLM

SEQ ID NO: 103 - protein, 168 aa, Homo sapiens ULBP4
HSLCFNFTIKSLSRPGQPWCEAQVFLNKNLFLQYNSDNNMVKPLGLLGKKVYATSTWGELTQTLGEVGRDLRMLLCDIKPQIKTSDPSTLQVEMFCQREAERCTGASWQFATNGEKSLLFDAMNMTWTVINHEASKIKETWKKDRGLEKYFRKLSKGDCDHWLREFLG

SEQ ID NO: 104 - protein, 169 aa, Homo sapiens ULBP5
HSLCYDITVIPKFRPGPRWCAVQGQVDEKTFLHYDCGSKTVTPVSPLGKKLNVTTAWKAQNPVLREVVDILTEQLLDIQLENYIPKEPLTLQARMSCEQKAEGHGSGSWQLSFDGQIFLLFDSENRMWTTVHPGARKMKEKWENDKDMTMSFHYISMGDCTGWLEDFLM

SEQ ID NO: 105 - protein, 169 aa, Homo sapiens ULBP6
HSLCYDITVIPKFRPGPRWCAVQGQVDEKTFLHYDCGNKTVTPVSPLGKKLNVTTAWKAQNPVLREVVDILTEQLLDIQLENYTPKEPLTLQARMSCEQKAEGHSSGSWQFSIDGQTFLLFDSEKRMWTTVHPGARKMKEKWENDKDVAMSFHYISMGDCIGWLEDFLM